European Patent Specification EP 3 377 897 B1, published May 1, 2024. Title: LACTATE BIOSENSORS AND USES THEREOF. Applicant: Duke University. The sequence listing filed with the application follows.

SEQUENCE LISTING (156 sequences)

SEQ ID NO: 1 - protein, 361 aa, Thermus thermophilus
MKRVSRRAFLRRLGVGVAATAAFSPLAVAQARRYRWRIQTAWDAGTVGYSLFQKFTERVKELTDGQLEVQPFPAGAVVGTFDMFDAVKTGVLDGMNPFTLYWAGRMPVTAFLSSYALGLDRPDQWETWFYSLGGLDIARRAFAEQGLFYVGPVQHDLNIIHSKKPIRRFEDFKGVKLRVPGGMIAEVFAAAGASTVLLPGGEVYPALERGVIDAADFVGPAVNYNLGFHQVAKYIIMGPPETPAIHQPVDLMDFTINLNRWRSLPKPLQERFIAAVHEYSWIHYAGIQKANLEAWPKYRQAGVEVIRLSNEDVRKFRRLAIPIWFKWAKMDKYSREAFASQLEYMKGIGYVTDEELKGLSL

SEQ ID NO: 2 - protein, 360 aa, Thermus scotoductus
MKENRRNFIRKLATGVAASSVFSPLAVAQAPRFRWRIQSAWDAGTVGYSLFQKFAERVKELTDGQIEIQTFPAGAVVGTFDMFDAVKTGVLDGMHPFTLYWAGRMPVTAFLSSYPLGLDRPDQWETWYYGLGGLELARKAYEEQGLFFVGPVQHDYNLIHSKKPIKSFEDFKGVKLRVPGGMIAEIFAAAGAATVLLPGGEVYPALERGVIDAADFVGPAVNYNLGFHQVTKYIIMGPPETPCIHQPVDLADITININRWRALPRNLQERFEAAVHEWSWIHYAGIQKANLETWPKYKAAGVQVIRLSTVDVRKFRRVAIPIWFKWAKQDKYTREAFASQLEYMKALGYVTDADIRGLSL

SEQ ID NO: 3 - protein, 360 aa, Thermus oshimai
MKSTRRQFLKKAAIGVAASSAFSPLAIAQAPRFRWRIQSAWDAGTVGYTLFQRFAERVKELTDGQIEIQPFPAGAVVGTFDMFDAVKTGVLDGMHPFTLYWAGRMPVTAFLSSYPLGLDRPDQWETWYYGLGGLELARKAYEEQGLAYIGPVQHDYNLIHSKKPIKSFEEFKGVKLRVPGGMIAEIFAAAGAATVLLPGGEVYPALERGVIDAADFVGPAVNYNLGFHQVTKYIIMGPPETPCIHQPVDLADITLNLNRWRAVPKNLQERFEAAVHEWSWVHYAGIQKANLEAWPKYRAAGVQIIRLSTVDVRKFRRVAIPIWFKWAKQDKYAKEAFQSQLEYMKALGYVTDVDLRGLSL

SEQ ID NO: 4 - protein, 386 aa, Thioalkalivibrio sulfidophilus
MSTKDDNGTGIVTGAAQEGSQTTSRRGFLKASAALGAGAILGAPYIGNAQTARGVRWRMQSAWQPGTIGYRTFETWCRSIQELTSGELSIEPFPAGAVAGTFEMADAVRSGVLDGMNWFTVYWPGKMPAGVFMSAYPMALSLPHHWDMMFDSFGGRQIVDELYDRQGLVFLGHVQHDLNLIHSKVPLRSFDDFRGKRIRFPGGIIAETFAKVGVRTTLLPGGDVYPALERGTIDAADFVGPAVNYDLGFHQVADYIIMGPPSTPCLHQPVDLMDISVNKRSWSRISEHTQKLMYKFVKAYSAEHFAAIQKANHEAWPKYKEAGVEVIHLSEEDAARFREAAIPLWFEWANKDRDAARLFKVHLEVMQDPSVAVITPDDIKDYKLNF

SEQ ID NO: 5 - protein, 366 aa, Roseobacter denitrificans
MTIKTTSRRNALRTLAGAGAATLAAPHIATAAGEGTTWKIQTSHTGGIGLATFKDWCSSIEEKTGGELAFTAFGANDVVGDFQLYDAVKNGVLDAVNPFTIYAQGIIPAATFLTSYPLGLRNPHEWDVFFYSLGGLEIARELYAAQGMKFVGPVHHGPNIIHSKVPIRSIDDFAGLKMRMPGGMVAEVFSEIGAETTVLPGSEIFPALEKGTIDAADFVGPAVNYALGFSQVTNYISMGPAGFMSLYQPVDLMDITVGQTAWDALSPQMQQFVEMETHVYSDMHHAAIQKADQEAWAKFEADGTEVTRLSQDDVELMTEVAVPIWFDYANRDKDAARVFKIQLDYMMSGSLGYVTPEQIEGLTLNL

SEQ ID NO: 6 - protein, 371 aa, Marinobacter
MTDITCKIETKGSARRRGFLKTLAVSAAISATLLASSVQAATTWKIQSVWDAGTVGYDLFKEWCDGMEEKTGGELKFTCFPAKAVAADNNGLFDAVRNGVLQGMNPFTLYWSGKIPASVFLSSYPAGPDQPHQWDTMFYSLGMLEKTREIYKKFGLFYVGPIQHDANIIHSKQPINSLDDLKGLKMRLPGGMVAEVFAKFGVAAVSLPGSDIFPALEKGTIDAADYVGPAVNWELGFSQVTKYILMGPPGIMSVYQPVDLMDLTVNLRAWNALDPKLQQIVEDEVRIYSQKHYLAIQKRNIEAMKKFEAAGTTVTRLSQEDLQEFRRAAIPIWYSWANKDEDAREIFDMQLEYMMNDTVGYITEDDIKGMN

SEQ ID NO: 7 - protein, 360 aa, Thermus sp.
MKETRRSFIRKVATGVAASAAFSPLAIAQAPRFRWRIQSAWDAGTVGYTLFQRFAERVKELTDGQIEIQTFPAGAVVGTFDMFDAVKTGVLDGMHPFTLYWAGRMPVTAFLSSYPLGLDRPDQWETWYYALGGLDLARRAFEEQGLFYVGPVQHDYNLIHSKKPIKSFEDFKGVKLRVPGGMIADVFSAAGAATVLLPGGEVYPALERGVIDAADFVGPAVNYNLGFHQVTKYIIMGPPETPCIHQPVDLADITLNLSRWRAVPKNLQERFEAAVHEWSWIHYAGIQKANLETWPKYKAAGVQIIRLTTVDVRKFRRVAIPIWFKWAKQDKYAREAFASQLEYMKALGYVTDADVRGLSL

SEQ ID NO: 8 - protein, 396 aa, Marinobacter adhaerens
MSACAGVAIDADKNKANGDVSMNSKNNIRNSCDTGETPPRRSFLKTIAMGATLAGAMLMGAGQAQAATTWKIQSTWDAGTVGYTLFEEWCKSIEAKSGGELKFQCFPAKAVAADNNALFDAVRNGVLQGMNPFTLYWAGKIPASVFLSSYPAGPDQPHQWDTMFYSMGMLEKTREIYKKFGLFYVGPIQHDANIIHSKQPVNSLDDLKGMKIRVPGGMVAEVFQQFGVSTVSLPGSDIFPALEKGTIDAADFVGPAVNYELGFSQVTDYIIFGPPGVMSIYQPVDLMDLTVSLRAWNSISPELQQLVEDEVRIYSQKHYLAIQARNIEAMEKFKADGDTVTRLSQEDLETWRKAAIPIWFNWANKNDDARAILDIQLKYMMNDTVGYITEEDIKGF

SEQ ID NO: 9 - protein, 387 aa, Anaeromyxobacter dehalogenans
MKKTTSRSQPDTAPKASRRSFLKKAALGAAGVAAGAAAPTIHVAQAPITLRFQSTWPQKDIFHEFALDYAKKVNEMSGGRLKIEVLAAGSVVKAFDLLDAVSKGTLDGGHGVVAYWYGKNTALALWGSGPAFGMDPNMVLAWHHYGGGRQLLEEIYRSLNLDVVSLMYGPMPTQPLGWFKQKPIAKPDDMKGLKFRTVGLSIDIFNGLGAAVNALPGAEIVPAMDRGLLDAAEFNNASSDRVLGFPDVSKICMLQSFHQCSEQFEILFNGKRFQALPADLKSIISIAAQAASADMSWKAIDRYSSDYFEMRDKQGVKFYSTRPEILKRQLEIWDQVMEKRAAENPTFKKVLESQRRFAQRAARWQNDTNVDFKMAYNHFFGGKKKAT

SEQ ID NO: 10 - protein, 343 aa, Polymorphum gilvum
MTEISRRGLLAGSVFGGVALAAPTVARAQEAVEWRMQALWDAGTTPFEFEKKFVERVGELTEGRFKITLYSAGQIVPANQAFDAVRSGAFEMMKTFDGYEAGKIPAFAFTSTIPFGFPQSDQYEAWFYELGGLDLAREAYAKGGLFYIAPTVYGEEPMHSTVKIESIADMAGKKGRFVGLASAVMADLGVAVSPLATAEVYTALEKGLIDFADRGDLTANYEAGLGEVAKFIILPGVHQPTTATSYVANQAAYQKLPDGFKAALAVAAREISGSLRQHILVQDMEVLTKYKDQGVEVVRLDAADIAAARAKAVESWEKATKGDELATRVLKGQVDFMTSLGLL

SEQ ID NO: 11 - protein, 365 aa, Pseudomonas stuztzeri
MKRRHLFGAAALLATLALAGCKDEQSQAPNQQAAGEPAKTYHWKMVTAWPKNYPGLGTSAERLAERVNAMSGGRLTIKVYAAGELVPALEVFDAVSRGTAELGHGASYYWKGKVPTAQFFTSVPFGLSTSEMNAWLSKGGGQAFWDEAYAPFGVKPLVIGNTGMQMGGWYNKEINSLTDLKGLKIRMPGLGGEVLSRLGATTVNLPGGEVFTALQTGAIDATDWVSPYNDLAFGLHKAARYYYYPGWQEPQAVLELLINQKAFDSLPADLQAIVTEASLAASRDMHDDYVYNNALALEQLKQQGTELKRFPDEVLAAMREQSDLILGELAAQSELNGRIWASMKAFQAQVEPMHEISEKELYNWR

SEQ ID NO: 12 - protein, 379 aa, Rhodobacter sphaeroides
MTAFEKKAAYSRRSFLRTGALAGGAAAGSVLAAPAVLAQAPLVMKMQTSWPASDIWMDFAREYVTRVEEMSGGRIKVDLLPAGAVVGAFQVMDAVHDGVIDASHSVSAYWYGKSKAASFFGTGPVFGGSATTMLGWFYQGGGQDLYRELTQDILGMNIVGFYGFPMPAQPFGWFKTEVNGVADIQGFKYRTVGLAADLLQAMGMSVAQLPGGEIVPAMERGVIDAFEFNNPSSDMRFGAQDVAKNYYLSSYHQASESFEYTFNRDFYEDLDPDLQAILKYAVEAASTSNTALALRQYSADLATLAAENGVAVHRTPKDILSGQLEAWDKLIVDLEADEFFKKVLDSQRAWVEQVSYYELMNAADLGLAYEHHFPGKLKL

SEQ ID NO: 13 - protein, 359 aa, Flexistipes sinusarabici
MGMMKKLLYSLLIILLVASAGFTAEKKIRWKLAMTWGPTLHPLSDTAEHMAEIVKELSDGNFVINIDASNVHKAPFGIFDMVKLGQYEMGHTASYYYKGKNIAFLPLTTMPFGMTAPEQYAWFYYGGGLELMQEAYTKHGMLAFPGGNTGNQMGGWFTKEINSLDDLKGLKMRIPGFAGQIMSKLGVTVTNIPPGELYTALERGTVDAVEWTGPGMDINMGFHKIAKYYYTGWHEPGSEVEFLINEKEYNKLPEKYKKILKIAMKTAAYDMYIQSYEMNAEAWQQMKEKYPDIKVKVFPEEVLKEMKTAYDNLVASYEKESPMFKKIMESKRAYLDKVRDWTHISDYLYLKSTSESNLN

SEQ ID NO: 14 - protein, 357 aa, Thermanaerovibrio acidaminovorans
MKRIKLLLTLCVALVALGALCGGALAAEEYKFKMATFYLKGDSAFDVIDHFRQLVWKKTGGKVRIDAFQAGELGFPVTEILEATSRGVVEMSIFYPNYKAAQDPVMALAGGRPGPMFDLRDQKAQVDATKDLLERSFGRFGVRYIAPMVYGEPEILVSRRPMSSLKDLKGRIFRASGMAAEFYTAIGAQAMMLPAGELYQALQLGTIDGLEWTDYTANYKLGFHEVAKNVLEPTKGVNLHSEATVHAFLVVNPKVWEKLPKEHQKAIQEACDEAYKWGADHLAKLNKTYKDKWIKAGAKVTQLPKEDQDKVIEVSAKILSGYSAKSPDAKEYCRRLVELWKKLGYTKWSDALAKQIK

SEQ ID NO: 15 - protein, 349 aa, Artificial Sequence
  ttLacPB1  (with signal peptide replaced with M and a GGSHHHHHH at C-terminus)
MFSPLAVAQARRYRWRIQTAWDAGTVGYSLFQKFTERVKELTDGQLEVQPFPAGAVVGTFDMFDAVKTGVLDGMNPFTLYWAGRMPVTAFLSSYALGLDRPDQWETWFYSLGGLDIARRAFAEQGLFYVGPVQHDLNIIHSKKPIRRFEDFKGVKLRVPGGMIAEVFAAAGASTVLLPGGEVYPALERGVIDAADFVGPAVNYNLGFHQVAKYIIMGPPETPAIHQPVDLMDFTINLNRWRSLPKPLQERFIAAVHEYSWIHYAGIQKANLEAWPKYRQAGVEVIRLSNEDVRKFRRLAIPIWFKWAKMDKYSREAFASQLEYMKGIGYVTDEELKGLSLGGSHHHHHH

SEQ ID NO: 16 - protein, 349 aa, Artificial Sequence
  tsLacBP2  (with signal peptide replaced with M and a GGSHHHHHH at C-terminus)
MFSPLAVAQAPRFRWRIQSAWDAGTVGYSLFQKFAERVKELTDGQIEIQTFPAGAVVGTFDMFDAVKTGVLDGMHPFTLYWAGRMPVTAFLSSYPLGLDRPDQWETWYYGLGGLELARKAYEEQGLFFVGPVQHDYNLIHSKKPIKSFEDFKGVKLRVPGGMIAEIFAAAGAATVLLPGGEVYPALERGVIDAADFVGPAVNYNLGFHQVTKYIIMGPPETPAIHQPVDLADITININRWRALPRNLQERFEAAVHEWSWIHYAGIQKANLETWPKYKAAGVQVIRLSTVDVRKFRRVAIPIWFKWAKQDKYTREAFASQLEYMKALGYVTDADIRGLSLGGSHHHHHH

SEQ ID NO: 17 - protein, 369 aa, Artificial Sequence
  toLacBP3  (with signal peptide replaced with M and a GGSHHHHHH at C-terminus)
MKSTRRQFLKKAAIGVAASSAFSPLAIAQAPRFRWRIQSAWDAGTVGYTLFQRFAERVKELTDGQIEIQPFPAGAVVGTFDMFDAVKTGVLDGMHPFTLYWAGRMPVTAFLSSYPLGLDRPDQWETWYYGLGGLELARKAYEEQGLAYIGPVQHDYNLIHSKKPIKSFEEFKGVKLRVPGGMIAEIFAAAGAATVLLPGGEVYPALERGVIDAADFVGPAVNYNLGFHQVTKYIIMGPPETPAIHQPVDLADITLNLNRWRAVPKNLQERFEAAVHEWSWVHYAGIQKANLEAWPKYRAAGVQIIRLSTVDVRKFRRVAIPIWFKWAKQDKYAKEAFQSQLEYMKALGYVTDVDLRGLSLGGSHHHHHH

SEQ ID NO: 18 - protein, 346 aa, Artificial Sequence
  tsLacBP4  (with signal peptide replaced with M and a GGSHHHHHH at C-terminus)
MTARGVRWRMQSAWQPGTIGYRTFETWARSIQELTSGELSIEPFPAGAVAGTFEMADAVRSGVLDGMNWFTVYWPGKMPAGVFMSAYPMALSLPHHWDMMFDSFGGRQIVDELYDRQGLVFLGHVQHDLNLIHSKVPLRSFDDFRGKRIRFPGGIIAETFAKVGVRTTLLPGGDVYPALERGTIDAADFVGPAVNYDLGFHQVADYIIMGPPSTPALHQPVDLMDISVNKRSWSRISEHTQKLMYKFVKAYSAEHFAAIQKANHEAWPKYKEAGVEVIHLSEEDAARFREAAIPLWFEWANKDRDAARLFKVHLEVMQDPSVAVITPDDIKDYKLNFGGSHHHHHH

SEQ ID NO: 19 - protein, 346 aa, Artificial Sequence
  rdLacBP5  (with signal peptide replaced with M and a GGSHHHHHH at C-terminus)
MAAGEGTTWKIQTSHTGGIGLATFKDWASSIEEKTGGELAFTAFGANDVVGDFQLYDAVKNGVLDAVNPFTIYAQGIIPAATFLTSYPLGLRNPHEWDVFFYSLGGLEIARELYAAQGMKFVGPVHHGPNIIHSKVPIRSIDDFAGLKMRMPGGMVAEVFSEIGAETTVLPGSEIFPALEKGTIDAADFVGPAVNYALGFSQVTNYISMGPAGFMSLYQPVDLMDITVGQTAWDALSPQMQQFVEMETHVYSDMHHAAIQKADQEAWAKFEADGTEVTRLSQDDVELMTEVAVPIWFDYANRDKDAARVFKIQLDYMMSGSLGYVTPEQIEGLTLNLGGSHHHHHH

SEQ ID NO: 20 - protein, 341 aa, Artificial Sequence
  msLacBP6  (with signal peptide replaced with M and a GGSHHHHHH at C-terminus)
MATTWKIQSVWDAGTVGYDLFKEWCDGMEEKTGGELKFTCFPAKAVAADNNGLFDAVRNGVLQGMNPFTLYWSGKIPASVFLSSYPAGPDQPHQWDTMFYSLGMLEKTREIYKKFGLFYVGPIQHDANIIHSKQPINSLDDLKGLKMRLPGGMVAEVFAKFGVAAVSLPGSDIFPALEKGTIDAADYVGPAVNWELGFSQVTKYILMGPPGIMSVYQPVDLMDLTVNLRAWNALDPKLQQIVEDEVRIYSQKHYLAIQKRNIEAMKKFEAAGTTVTRLSQEDLQEFRRAAIPIWYSWANKDEDAREIFDMQLEYMMNDTVGYITEDDIKGMNGGSHHHHHH

SEQ ID NO: 21 - protein, 342 aa, Artificial Sequence
  tsLacBP7  (with signal peptide replaced with M and a GGSHHHHHH at C-terminus)
MQAPRFRWRIQSAWDAGTVGYTLFQRFAERVKELTDGQIEIQTFPAGAVVGTFDMFDAVKTGVLDGMHPFTLYWAGRMPVTAFLSSYPLGLDRPDQWETWYYALGGLDLARRAFEEQGLFYVGPVQHDYNLIHSKKPIKSFEDFKGVKLRVPGGMIADVFSAAGAATVLLPGGEVYPALERGVIDAADFVGPAVNYNLGFHQVTKYIIMGPPETPAIHQPVDLADITLNLSRWRAVPKNLQERFEAAVHEWSWIHYAGIQKANLETWPKYKAAGVQIIRLTTVDVRKFRRVAIPIWFKWAKQDKYAREAFASQLEYMKALGYVTDADVRGLSLGGSHHHHHH

SEQ ID NO: 22 - protein, 342 aa, Artificial Sequence
  maLacBP8  (with signal peptide replaced with M and a GGSHHHHHH at C-terminus)
MQAATTWKIQSTWDAGTVGYTLFEEWAKSIEAKSGGELKFQAFPAKAVAADNNALFDAVRNGVLQGMNPFTLYWAGKIPASVFLSSYPAGPDQPHQWDTMFYSMGMLEKTREIYKKFGLFYVGPIQHDANIIHSKQPVNSLDDLKGMKIRVPGGMVAEVFQQFGVSTVSLPGSDIFPALEKGTIDAADFVGPAVNYELGFSQVTDYIIFGPPGVMSIYQPVDLMDLTVSLRAWNSISPELQQLVEDEVRIYSQKHYLAIQARNIEAMEKFKADGDTVTRLSQEDLETWRKAAIPIWFNWANKNDDARAILDIQLKYMMNDTVGYITEEDIKGFGGSHHHHHH

SEQ ID NO: 23 - protein, 353 aa, Artificial Sequence
  adLacBP9  (with signal peptide replaced with M and a GGSHHHHHH at C-terminus)
MQAPITLRFQSTWPQKDIFHEFALDYAKKVNEMSGGRLKIEVLAAGSVVKAFDLLDAVSKGTLDGGHGVVAYWYGKNTALALWGSGPAFGMDPNMVLAWHHYGGGRQLLEEIYRSLNLDVVSLMYGPMPTQPLGWFKQKPIAKPDDMKGLKFRTVGLSIDIFNGLGAAVNALPGAEIVPAMDRGLLDAAEFNNASSDRVLGFPDVSKIAMLQSFHQASEQFEILFNGKRFQALPADLKSIISIAAQAASADMSWKAIDRYSSDYFEMRDKQGVKFYSTRPEILKRQLEIWDQVMEKRAAENPTFKKVLESQRRFAQRAARWQNDTNVDFKMAYNHFFGGKKKATGGSHHHHHH

SEQ ID NO: 24 - protein, 325 aa, Artificial Sequence
  pgLacBP10  (with signal peptide replaced with M and a GGSHHHHHH at C-terminus)
MQEAVEWRMQALWDAGTTPFEFEKKFVERVGELTEGRFKITLYSAGQIVPANQAFDAVRSGAFEMMKTFDGYEAGKIPAFAFTSTIPFGFPQSDQYEAWFYELGGLDLAREAYAKGGLFYIAPTVYGEEPMHSTVKIESIADMAGKKGRFVGLASAVMADLGVAVSPLATAEVYTALEKGLIDFADRGDLTANYEAGLGEVAKFIILPGVHQPTTATSYVANQAAYQKLPDGFKAALAVAAREISGSLRQHILVQDMEVLTKYKDQGVEVVRLDAADIAAARAKAVESWEKATKGDELATRVLKGQVDFMTSLGLLGGSHHHHHH

SEQ ID NO: 25 - protein, 345 aa, Artificial Sequence
  psLacBP11  (with signal peptide replaced with M and a GGSHHHHHH at C-terminus)
MQQAAGEPAKTYHWKMVTAWPKNYPGLGTSAERLAERVNAMSGGRLTIKVYAAGELVPALEVFDAVSRGTAELGHGASYYWKGKVPTAQFFTSVPFGLSTSEMNAWLSKGGGQAFWDEAYAPFGVKPLVIGNTGMQMGGWYNKEINSLTDLKGLKIRMPGLGGEVLSRLGATTVNLPGGEVFTALQTGAIDATDWVSPYNDLAFGLHKAARYYYYPGWQEPQAVLELLINQKAFDSLPADLQAIVTEASLAASRDMHDDYVYNNALALEQLKQQGTELKRFPDEVLAAMREQSDLILGELAAQSELNGRIWASMKAFQAQVEPMHEISEKELYNWRGGSHHHHHH

SEQ ID NO: 26 - protein, 350 aa, Artificial Sequence
  rsLacBP12 (with signal peptide replaced with M and a GGSHHHHHH at C-terminus)
MQAPLVMKMQTSWPASDIWMDFAREYVTRVEEMSGGRIKVDLLPAGAVVGAFQVMDAVHDGVIDASHSVSAYWYGKSKAASFFGTGPVFGGSATTMLGWFYQGGGQDLYRELTQDILGMNIVGFYGFPMPAQPFGWFKTEVNGVADIQGFKYRTVGLAADLLQAMGMSVAQLPGGEIVPAMERGVIDAFEFNNPSSDMRFGAQDVAKNYYLSSYHQASESFEYTFNRDFYEDLDPDLQAILKYAVEAASTSNTALALRQYSADLATLAAENGVAVHRTPKDILSGQLEAWDKLIVDLEADEFFKKVLDSQRAWVEQVSYYELMNAADLGLAYEHHFPGKLKLGGSHHHHH

SEQ ID NO: 27 - protein, 345 aa, Artificial Sequence
  fsLacBP13  (with signal peptide replaced with M and a GGSHHHHHH at C-terminus)
MEKKIRWKLAMTWGPTLHPLSDTAEHMAEIVKELSDGNFVINIDASNVHKAPFGIFDMVKLGQYEMGHTASYYYKGKNIAFLPLTTMPFGMTAPEQYAWFYYGGGLELMQEAYTKHGMLAFPGGNTGNQMGGWFTKEINSLDDLKGLKMRIPGFAGQIMSKLGVTVTNIPPGELYTALERGTVDAVEWTGPGMDINMGFHKIAKYYYTGWHEPGSEVEFLINEKEYNKLPEKYKKILKIAMKTAAYDMYIQSYEMNAEAWQQMKEKYPDIKVKVFPEEVLKEMKTAYDNLVASYEKESPMFKKIMESKRAYLDKVRDWTHISDYLYLKSTSESNLNGGSHHHHHH

SEQ ID NO: 28 - protein, 340 aa, Artificial Sequence
  taLacBP14  (with signal peptide replaced with M and a GGSHHHHHH at C-terminus)
MEEYKFKMATFYLKGDSAFDVIDHFRQLVWKKTGGKVRIDAFQAGELGFPVTEILEATSRGVVEMSIFYPNYKAAQDPVMALAGGRPGPMFDLRDQKAQVDATKDLLERSFGRFGVRYIAPMVYGEPEILVSRRPMSSLKDLKGRIFRASGMAAEFYTAIGAQAMMLPAGELYQALQLGTIDGLEWTDYTANYKLGFHEVAKNVLEPTKGVNLHSEATVHAFLVVNPKVWEKLPKEHQKAIQEAADEAYKWGADHLAKLNKTYKDKWIKAGAKVTQLPKEDQDKVIEVSAKILSGYSAKSPDAKEYARRLVELWKKLGYTKWSDALAKQIKGGSHHHHHH

SEQ ID NO: 29 - protein, 341 aa, Artificial Sequence
  msLacBP6.10C (10C substitution mutant with signal peptide replaced with M and a GGSHHHHHH at C-terminus)
MATTWKIQSCWDAGTVGYDLFKEWSDGMEEKTGGELKFTAFPAKAVAADNNGLFDAVRNGVLQGMNPFTLYWSGKIPASVFLSSYPAGPDQPHQWDTMFYSLGMLEKTREIYKKFGLFYVGPIQHDANIIHSKQPINSLDDLKGLKMRLPGGMVAEVFAKFGVAAVSLPGSDIFPALEKGTIDAADYVGPAVNWELGFSQVTKYILMGPPGIMSVYQPVDLMDLTVNLRAWNALDPKLQQIVEDEVRIYSQKHYLAIQKRNIEAMKKFEAAGTTVTRLSQEDLQEFRRAAIPIWYSWANKDEDAREIFDMQLEYMMNDTVGYITEDDIKGMNGGSHHHHHH

SEQ ID NO: 30 - protein, 341 aa, Artificial Sequence
  msLacBP6.12C (12C substitution mutant with signal peptide replaced with M and a GGSHHHHHH at C-terminus)
MATTWKIQSVWCAGTVGYDLFKEWSDGMEEKTGGELKFTAFPAKAVAADNNGLFDAVRNGVLQGMNPFTLYWSGKIPASVFLSSYPAGPDQPHQWDTMFYSLGMLEKTREIYKKFGLFYVGPIQHDANIIHSKQPINSLDDLKGLKMRLPGGMVAEVFAKFGVAAVSLPGSDIFPALEKGTIDAADYVGPAVNWELGFSQVTKYILMGPPGIMSVYQPVDLMDLTVNLRAWNALDPKLQQIVEDEVRIYSQKHYLAIQKRNIEAMKKFEAAGTTVTRLSQEDLQEFRRAAIPIWYSWANKDEDAREIFDMQLEYMMNDTVGYITEDDIKGMNGGSHHHHHH

SEQ ID NO: 31 - protein, 341 aa, Artificial Sequence
  msLacBP6.43C (43C substitution mutant with signal peptide replaced with M and a GGSHHHHHH at C-terminus)
MATTWKIQSVWDAGTVGYDLFKEWSDGMEEKTGGELKFTAFPCKAVAADNNGLFDAVRNGVLQGMNPFTLYWSGKIPASVFLSSYPAGPDQPHQWDTMFYSLGMLEKTREIYKKFGLFYVGPIQHDANIIHSKQPINSLDDLKGLKMRLPGGMVAEVFAKFGVAAVSLPGSDIFPALEKGTIDAADYVGPAVNWELGFSQVTKYILMGPPGIMSVYQPVDLMDLTVNLRAWNALDPKLQQIVEDEVRIYSQKHYLAIQKRNIEAMKKFEAAGTTVTRLSQEDLQEFRRAAIPIWYSWANKDEDAREIFDMQLEYMMNDTVGYITEDDIKGMNGGSHHHHHH

SEQ ID NO: 32 - protein, 341 aa, Artificial Sequence
  msLacBP6.49C (49C substitution mutant with signal peptide replaced with M and a GGSHHHHHH at C-terminus)
MATTWKIQSVWDAGTVGYDLFKEWSDGMEEKTGGELKFTAFPAKAVAACNNGLFDAVRNGVLQGMNPFTLYWSGKIPASVFLSSYPAGPDQPHQWDTMFYSLGMLEKTREIYKKFGLFYVGPIQHDANIIHSKQPINSLDDLKGLKMRLPGGMVAEVFAKFGVAAVSLPGSDIFPALEKGTIDAADYVGPAVNWELGFSQVTKYILMGPPGIMSVYQPVDLMDLTVNLRAWNALDPKLQQIVEDEVRIYSQKHYLAIQKRNIEAMKKFEAAGTTVTRLSQEDLQEFRRAAIPIWYSWANKDEDAREIFDMQLEYMMNDTVGYITEDDIKGMNGGSHHHHHH

SEQ ID NO: 33 - protein, 341 aa, Artificial Sequence
  msLacBP6.50C  (50C substitution mutant with signal peptide replaced with M and a GGSHHHHHH at C-terminus)
MATTWKIQSVWDAGTVGYDLFKEWSDGMEEKTGGELKFTAFPAKAVAADCNGLFDAVRNGVLQGMNPFTLYWSGKIPASVFLSSYPAGPDQPHQWDTMFYSLGMLEKTREIYKKFGLFYVGPIQHDANIIHSKQPINSLDDLKGLKMRLPGGMVAEVFAKFGVAAVSLPGSDIFPALEKGTIDAADYVGPAVNWELGFSQVTKYILMGPPGIMSVYQPVDLMDLTVNLRAWNALDPKLQQIVEDEVRIYSQKHYLAIQKRNIEAMKKFEAAGTTVTRLSQEDLQEFRRAAIPIWYSWANKDEDAREIFDMQLEYMMNDTVGYITEDDIKGMNGGSHHHHHH

SEQ ID NO: 34 - protein, 341 aa, Artificial Sequence
  msLacBP6.68C  (68C substitution mutant with signal peptide replaced with M and a GGSHHHHHH at C-terminus)
MATTWKIQSVWDAGTVGYDLFKEWSDGMEEKTGGELKFTAFPAKAVAADNNGLFDAVRNGVLQGMNPCTLYWSGKIPASVFLSSYPAGPDQPHQWDTMFYSLGMLEKTREIYKKFGLFYVGPIQHDANIIHSKQPINSLDDLKGLKMRLPGGMVAEVFAKFGVAAVSLPGSDIFPALEKGTIDAADYVGPAVNWELGFSQVTKYILMGPPGIMSVYQPVDLMDLTVNLRAWNALDPKLQQIVEDEVRIYSQKHYLAIQKRNIEAMKKFEAAGTTVTRLSQEDLQEFRRAAIPIWYSWANKDEDAREIFDMQLEYMMNDTVGYITEDDIKGMNGGSHHHHHH

SEQ ID NO: 35 - protein, 341 aa, Artificial Sequence
  msLacBP6.169C  (169C substitution mutant with signal peptide replaced with M and a GGSHHHHHH at C-terminus)
MATTWKIQSVWDAGTVGYDLFKEWSDGMEEKTGGELKFTAFPAKAVAADNNGLFDAVRNGVLQGMNPFTLYWSGKIPASVFLSSYPAGPDQPHQWDTMFYSLGMLEKTREIYKKFGLFYVGPIQHDANIIHSKQPINSLDDLKGLKMRLPGGMVAEVFAKFGVAAVSLCGSDIFPALEKGTIDAADYVGPAVNWELGFSQVTKYILMGPPGIMSVYQPVDLMDLTVNLRAWNALDPKLQQIVEDEVRIYSQKHYLAIQKRNIEAMKKFEAAGTTVTRLSQEDLQEFRRAAIPIWYSWANKDEDAREIFDMQLEYMMNDTVGYITEDDIKGMNGGSHHHHHH

SEQ ID NO: 36 - protein, 341 aa, Artificial Sequence
  msLacBP6.170C  (170C substitution mutant with signal peptide replaced with M and a GGSHHHHHH at C-terminus)
MATTWKIQSVWDAGTVGYDLFKEWSDGMEEKTGGELKFTAFPAKAVAADNNGLFDAVRNGVLQGMNPFTLYWSGKIPASVFLSSYPAGPDQPHQWDTMFYSLGMLEKTREIYKKFGLFYVGPIQHDANIIHSKQPINSLDDLKGLKMRLPGGMVAEVFAKFGVAAVSLPCSDIFPALEKGTIDAADYVGPAVNWELGFSQVTKYILMGPPGIMSVYQPVDLMDLTVNLRAWNALDPKLQQIVEDEVRIYSQKHYLAIQKRNIEAMKKFEAAGTTVTRLSQEDLQEFRRAAIPIWYSWANKDEDAREIFDMQLEYMMNDTVGYITEDDIKGMNGGSHHHHHH

SEQ ID NO: 37 - protein, 341 aa, Artificial Sequence
  msLacBP6.171C  (171C substitution mutant with signal peptide replaced with M and a GGSHHHHHH at C-terminus)
MATTWKIQSVWDAGTVGYDLFKEWSDGMEEKTGGELKFTAFPAKAVAADNNGLFDAVRNGVLQGMNPFTLYWSGKIPASVFLSSYPAGPDQPHQWDTMFYSLGMLEKTREIYKKFGLFYVGPIQHDANIIHSKQPINSLDDLKGLKMRLPGGMVAEVFAKFGVAAVSLPGCDIFPALEKGTIDAADYVGPAVNWELGFSQVTKYILMGPPGIMSVYQPVDLMDLTVNLRAWNALDPKLQQIVEDEVRIYSQKHYLAIQKRNIEAMKKFEAAGTTVTRLSQEDLQEFRRAAIPIWYSWANKDEDAREIFDMQLEYMMNDTVGYITEDDIKGMNGGSHHHHHH

SEQ ID NO: 38 - protein, 341 aa, Artificial Sequence
  msLacBP6.187C  (187C substitution mutant with signal peptide replaced with M and a GGSHHHHHH at C-terminus)
MATTWKIQSVWDAGTVGYDLFKEWSDGMEEKTGGELKFTAFPAKAVAADNNGLFDAVRNGVLQGMNPFTLYWSGKIPASVFLSSYPAGPDQPHQWDTMFYSLGMLEKTREIYKKFGLFYVGPIQHDANIIHSKQPINSLDDLKGLKMRLPGGMVAEVFAKFGVAAVSLPGSDIFPALEKGTIDAADCVGPAVNWELGFSQVTKYILMGPPGIMSVYQPVDLMDLTVNLRAWNALDPKLQQIVEDEVRIYSQKHYLAIQKRNIEAMKKFEAAGTTVTRLSQEDLQEFRRAAIPIWYSWANKDEDAREIFDMQLEYMMNDTVGYITEDDIKGMNGGSHHHHHH

SEQ ID NO: 39 - protein, 341 aa, Artificial Sequence
  msLacBP6.188C  (188C substitution mutant with signal peptide replaced with M and a GGSHHHHHH at C-terminus)
MATTWKIQSVWDAGTVGYDLFKEWSDGMEEKTGGELKFTAFPAKAVAADNNGLFDAVRNGVLQGMNPFTLYWSGKIPASVFLSSYPAGPDQPHQWDTMFYSLGMLEKTREIYKKFGLFYVGPIQHDANIIHSKQPINSLDDLKGLKMRLPGGMVAEVFAKFGVAAVSLPGSDIFPALEKGTIDAADYCGPAVNWELGFSQVTKYILMGPPGIMSVYQPVDLMDLTVNLRAWNALDPKLQQIVEDEVRIYSQKHYLAIQKRNIEAMKKFEAAGTTVTRLSQEDLQEFRRAAIPIWYSWANKDEDAREIFDMQLEYMMNDTVGYITEDDIKGMNGGSHHHHHH

SEQ ID NO: 40 - protein, 341 aa, Artificial Sequence
  msLacBP6.192C  (192C substitution mutant with signal peptide replaced with M and a GGSHHHHHH at C-terminus)
MATTWKIQSVWDAGTVGYDLFKEWSDGMEEKTGGELKFTAFPAKAVAADNNGLFDAVRNGVLQGMNPFTLYWSGKIPASVFLSSYPAGPDQPHQWDTMFYSLGMLEKTREIYKKFGLFYVGPIQHDANIIHSKQPINSLDDLKGLKMRLPGGMVAEVFAKFGVAAVSLPGSDIFPALEKGTIDAADYVGPACNWELGFSQVTKYILMGPPGIMSVYQPVDLMDLTVNLRAWNALDPKLQQIVEDEVRIYSQKHYLAIQKRNIEAMKKFEAAGTTVTRLSQEDLQEFRRAAIPIWYSWANKDEDAREIFDMQLEYMMNDTVGYITEDDIKGMNGGSHHHHHH

SEQ ID NO: 41 - protein, 341 aa, Artificial Sequence
  msLacBP6.196C  (196C substitution mutant with signal peptide replaced with M and a GGSHHHHHH at C-terminus)
MATTWKIQSVWDAGTVGYDLFKEWSDGMEEKTGGELKFTAFPAKAVAADNNGLFDAVRNGVLQGMNPFTLYWSGKIPASVFLSSYPAGPDQPHQWDTMFYSLGMLEKTREIYKKFGLFYVGPIQHDANIIHSKQPINSLDDLKGLKMRLPGGMVAEVFAKFGVAAVSLPGSDIFPALEKGTIDAADYVGPAVNWECGFSQVTKYILMGPPGIMSVYQPVDLMDLTVNLRAWNALDPKLQQIVEDEVRIYSQKHYLAIQKRNIEAMKKFEAAGTTVTRLSQEDLQEFRRAAIPIWYSWANKDEDAREIFDMQLEYMMNDTVGYITEDDIKGMNGGSHHHHHH

SEQ ID NO: 42 - protein, 342 aa, Artificial Sequence
  tsLacBP7.189C  (189C substitution mutant with signal peptide replaced with M and a GGSHHHHHH at C-terminus)
MQAPRFRWRIQSAWDAGTVGYTLFQRFAERVKELTDGQIEIQTFPAGAVVGTFDMFDAVKTGVLDGMHPFTLYWAGRMPVTAFLSSYPLGLDRPDQWETWYYALGGLDLARRAFEEQGLFYVGPVQHDYNLIHSKKPIKSFEDFKGVKLRVPGGMIADVFSAAGAATVLLPGGEVYPALERGVIDAADCVGPAVNYNLGFHQVTKYIIMGPPETPAIHQPVDLADITLNLSRWRAVPKNLQERFEAAVHEWSWIHYAGIQKANLETWPKYKAAGVQIIRLTTVDVRKFRRVAIPIWFKWAKQDKYAREAFASQLEYMKALGYVTDADVRGLSLGGSHHHHHH

SEQ ID NO: 43 - protein, 342 aa, Artificial Sequence
  maLacBP8.189C  (189C substitution mutant with signal peptide replaced with M and a GGSHHHHHH at C-terminus)
MQAATTWKIQSTWDAGTVGYTLFEEWAKSIEAKSGGELKFQAFPAKAVAADNNALFDAVRNGVLQGMNPFTLYWAGKIPASVFLSSYPAGPDQPHQWDTMFYSMGMLEKTREIYKKFGLFYVGPIQHDANIIHSKQPVNSLDDLKGMKIRVPGGMVAEVFQQFGVSTVSLPGSDIFPALEKGTIDAADCVGPAVNYELGFSQVTDYIIFGPPGVMSIYQPVDLMDLTVSLRAWNSISPELQQLVEDEVRIYSQKHYLAIQARNIEAMEKFKADGDTVTRLSQEDLETWRKAAIPIWFNWANKNDDARAILDIQLKYMMNDTVGYITEEDIKGFGGSHHHHHH

SEQ ID NO: 44 - protein, 353 aa, Artificial Sequence
  adLacBP9.C191  (191C substitution mutant with signal peptide replaced with M and a GGSHHHHHH at C-terminus)
MQAPITLRFQSTWPQKDIFHEFALDYAKKVNEMSGGRLKIEVLAAGSVVKAFDLLDAVSKGTLDGGHGVVAYWYGKNTALALWGSGPAFGMDPNMVLAWHHYGGGRQLLEEIYRSLNLDVVSLMYGPMPTQPLGWFKQKPIAKPDDMKGLKFRTVGLSIDIFNGLGAAVNALPGAEIVPAMDRGLLDAAECNNASSDRVLGFPDVSKIAMLQSFHQASEQFEILFNGKRFQALPADLKSIISIAAQAASADMSWKAIDRYSSDYFEMRDKQGVKFYSTRPEILKRQLEIWDQVMEKRAAENPTFKKVLESQRRFAQRAARWQNDTNVDFKMAYNHFFGGKKKATGGSHHHHHH

SEQ ID NO: 45 - protein, 345 aa, Artificial Sequence
  psLacBP11.195C  (195C substitution mutant with signal peptide replaced with M and a GGSHHHHHH at C-terminus)
MQQAAGEPAKTYHWKMVTAWPKNYPGLGTSAERLAERVNAMSGGRLTIKVYAAGELVPALEVFDAVSRGTAELGHGASYYWKGKVPTAQFFTSVPFGLSTSEMNAWLSKGGGQAFWDEAYAPFGVKPLVIGNTGMQMGGWYNKEINSLTDLKGLKIRMPGLGGEVLSRLGATTVNLPGGEVFTALQTGAIDATDCVSPYNDLAFGLHKAARYYYYPGWQEPQAVLELLINQKAFDSLPADLQAIVTEASLAASRDMHDDYVYNNALALEQLKQQGTELKRFPDEVLAAMREQSDLILGELAAQSELNGRIWASMKAFQAQVEPMHEISEKELYNWRGGSHHHHHH

SEQ ID NO: 46 - protein, 351 aa, Artificial Sequence
  rsLacBP12.191C  (191C substitution mutant with signal peptide replaced with M and a GGSHHHHHH at C-terminus)
MQAPLVMKMQTSWPASDIWMDFAREYVTRVEEMSGGRIKVDLLPAGAVVGAFQVMDAVHDGVIDASHSVSAYWYGKSKAASFFGTGPVFGGSATTMLGWFYQGGGQDLYRELTQDILGMNIVGFYGFPMPAQPFGWFKTEVNGVADIQGFKYRTVGLAADLLQAMGMSVAQLPGGEIVPAMERGVIDAFECNNPSSDMRFGAQDVAKNYYLSSYHQASESFEYTFNRDFYEDLDPDLQAILKYAVEAASTSNTALALRQYSADLATLAAENGVAVHRTPKDILSGQLEAWDKLIVDLEADEFFKKVLDSQRAWVEQVSYYELMNAADLGLAYEHHFPGKLKLGGSHHHHHH

SEQ ID NO: 47 - protein, 345 aa, Artificial Sequence
  fsLacBP13.188C  (188C substitution mutant with signal peptide replaced with M and a GGSHHHHHH at C-terminus)
MEKKIRWKLAMTWGPTLHPLSDTAEHMAEIVKELSDGNFVINIDASNVHKAPFGIFDMVKLGQYEMGHTASYYYKGKNIAFLPLTTMPFGMTAPEQYAWFYYGGGLELMQEAYTKHGMLAFPGGNTGNQMGGWFTKEINSLDDLKGLKMRIPGFAGQIMSKLGVTVTNIPPGELYTALERGTVDAVECTGPGMDINMGFHKIAKYYYTGWHEPGSEVEFLINEKEYNKLPEKYKKILKIAMKTAAYDMYIQSYEMNAEAWQQMKEKYPDIKVKVFPEEVLKEMKTAYDNLVASYEKESPMFKKIMESKRAYLDKVRDWTHISDYLYLKSTSESNLNGGSHHHHHH

SEQ ID NO: 48 - protein, 340 aa, Artificial Sequence
  taLacBP14.186C  (186C substitution mutant with signal peptide replaced with M and a GGSHHHHHH at C-terminus)
MEEYKFKMATFYLKGDSAFDVIDHFRQLVWKKTGGKVRIDAFQAGELGFPVTEILEATSRGVVEMSIFYPNYKAAQDPVMALAGGRPGPMFDLRDQKAQVDATKDLLERSFGRFGVRYIAPMVYGEPEILVSRRPMSSLKDLKGRIFRASGMAAEFYTAIGAQAMMLPAGELYQALQLGTIDGLECTDYTANYKLGFHEVAKNVLEPTKGVNLHSEATVHAFLVVNPKVWEKLPKEHQKAIQEAADEAYKWGADHLAKLNKTYKDKWIKAGAKVTQLPKEDQDKVIEVSAKILSGYSAKSPDAKEYARRLVELWKKLGYTKWSDALAKQIKGGSHHHHHH

SEQ ID NO: 49 - protein, 341 aa, Artificial Sequence
  msLacBP6_187C_F68L (187C, 68L double substitution mutant with signal peptide replaced with M and a GGSHHHHHH at C-terminus)
MATTWKIQSVWDAGTVGYDLFKEWCDGMEEKTGGELKFTCFPAKAVAADNNGLFDAVRNGVLQGMNPLTLYWSGKIPASVFLSSYPAGPDQPHQWDTMFYSLGMLEKTREIYKKFGLFYVGPIQHDANIIHSKQPINSLDDLKGLKMRLPGGMVAEVFAKFGVAAVSLPGSDIFPALEKGTIDAADCVGPAVNWELGFSQVTKYILMGPPGIMSVYQPVDLMDLTVNLRAWNALDPKLQQIVEDEVRIYSQKHYLAIQKRNIEAMKKFEAAGTTVTRLSQEDLQEFRRAAIPIWYSWANKDEDAREIFDMQLEYMMNDTVGYITEDDIKGMNGGSHHHHHH

SEQ ID NO: 50 - protein, 341 aa, Artificial Sequence
  msLacBP6_187C_F68M (187C, 68M double substitution mutant with signal peptide replaced with M and a GGSHHHHHH at C-terminus)
MATTWKIQSVWDAGTVGYDLFKEWCDGMEEKTGGELKFTCFPAKAVAADNNGLFDAVRNGVLQGMNPMTLYWSGKIPASVFLSSYPAGPDQPHQWDTMFYSLGMLEKTREIYKKFGLFYVGPIQHDANIIHSKQPINSLDDLKGLKMRLPGGMVAEVFAKFGVAAVSLPGSDIFPALEKGTIDAADCVGPAVNWELGFSQVTKYILMGPPGIMSVYQPVDLMDLTVNLRAWNALDPKLQQIVEDEVRIYSQKHYLAIQKRNIEAMKKFEAAGTTVTRLSQEDLQEFRRAAIPIWYSWANKDEDAREIFDMQLEYMMNDTVGYITEDDIKGMNGGSHHHHHH

SEQ ID NO: 51 - protein, 341 aa, Artificial Sequence
  msLacBP6_187C_L70F  (187C, 70F double substitution mutant with signal peptide replaced with M and a GGSHHHHHH at C-terminus)
MATTWKIQSVWDAGTVGYDLFKEWCDGMEEKTGGELKFTCFPAKAVAADNNGLFDAVRNGVLQGMNPFTFYWSGKIPASVFLSSYPAGPDQPHQWDTMFYSLGMLEKTREIYKKFGLFYVGPIQHDANIIHSKQPINSLDDLKGLKMRLPGGMVAEVFAKFGVAAVSLPGSDIFPALEKGTIDAADCVGPAVNWELGFSQVTKYILMGPPGIMSVYQPVDLMDLTVNLRAWNALDPKLQQIVEDEVRIYSQKHYLAIQKRNIEAMKKFEAAGTTVTRLSQEDLQEFRRAAIPIWYSWANKDEDAREIFDMQLEYMMNDTVGYITEDDIKGMNGGSHHHHHH

SEQ ID NO: 52 - protein, 341 aa, Artificial Sequence
  msLacBP6_187C_L70I  (187C, 70I double substitution mutant with signal peptide replaced with M and a GGSHHHHHH at C-terminus)
MATTWKIQSVWDAGTVGYDLFKEWCDGMEEKTGGELKFTCFPAKAVAADNNGLFDAVRNGVLQGMNPFTIYWSGKIPASVFLSSYPAGPDQPHQWDTMFYSLGMLEKTREIYKKFGLFYVGPIQHDANIIHSKQPINSLDDLKGLKMRLPGGMVAEVFAKFGVAAVSLPGSDIFPALEKGTIDAADCVGPAVNWELGFSQVTKYILMGPPGIMSVYQPVDLMDLTVNLRAWNALDPKLQQIVEDEVRIYSQKHYLAIQKRNIEAMKKFEAAGTTVTRLSQEDLQEFRRAAIPIWYSWANKDEDAREIFDMQLEYMMNDTVGYITEDDIKGMNGGSHHHHHH

SEQ ID NO: 53 - protein, 341 aa, Artificial Sequence
  msLacBP6_187C_L70M  (187C, 70M double substitution mutant with signal peptide replaced with M and a GGSHHHHHH at C-terminus)
MATTWKIQSVWDAGTVGYDLFKEWCDGMEEKTGGELKFTCFPAKAVAADNNGLFDAVRNGVLQGMNPFTMYWSGKIPASVFLSSYPAGPDQPHQWDTMFYSLGMLEKTREIYKKFGLFYVGPIQHDANIIHSKQPINSLDDLKGLKMRLPGGMVAEVFAKFGVAAVSLPGSDIFPALEKGTIDAADCVGPAVNWELGFSQVTKYILMGPPGIMSVYQPVDLMDLTVNLRAWNALDPKLQQIVEDEVRIYSQKHYLAIQKRNIEAMKKFEAAGTTVTRLSQEDLQEFRRAAIPIWYSWANKDEDAREIFDMQLEYMMNDTVGYITEDDIKGMNGGSHHHHHH

SEQ ID NO: 54 - protein, 341 aa, Artificial Sequence
  msLacBP6_187C_P150A  (187C, 150A double substitution mutant with signal peptide replaced with M and a GGSHHHHHH at C-terminus)
MATTWKIQSVWDAGTVGYDLFKEWCDGMEEKTGGELKFTCFPAKAVAADNNGLFDAVRNGVLQGMNPFTLYWSGKIPASVFLSSYPAGPDQPHQWDTMFYSLGMLEKTREIYKKFGLFYVGPIQHDANIIHSKQPINSLDDLKGLKMRLAGGMVAEVFAKFGVAAVSLPGSDIFPALEKGTIDAADCVGPAVNWELGFSQVTKYILMGPPGIMSVYQPVDLMDLTVNLRAWNALDPKLQQIVEDEVRIYSQKHYLAIQKRNIEAMKKFEAAGTTVTRLSQEDLQEFRRAAIPIWYSWANKDEDAREIFDMQLEYMMNDTVGYITEDDIKGMNGGSHHHHHH

SEQ ID NO: 55 - protein, 341 aa, Artificial Sequence
  msLacBP6_187C_P150S  (187C, 150S double substitution mutant with signal peptide replaced with M and a GGSHHHHHH at C-terminus)
MATTWKIQSVWDAGTVGYDLFKEWCDGMEEKTGGELKFTCFPAKAVAADNNGLFDAVRNGVLQGMNPFTLYWSGKIPASVFLSSYPAGPDQPHQWDTMFYSLGMLEKTREIYKKFGLFYVGPIQHDANIIHSKQPINSLDDLKGLKMRLSGGMVAEVFAKFGVAAVSLPGSDIFPALEKGTIDAADCVGPAVNWELGFSQVTKYILMGPPGIMSVYQPVDLMDLTVNLRAWNALDPKLQQIVEDEVRIYSQKHYLAIQKRNIEAMKKFEAAGTTVTRLSQEDLQEFRRAAIPIWYSWANKDEDAREIFDMQLEYMMNDTVGYITEDDIKGMNGGSHHHHHH

SEQ ID NO: 56 - protein, 341 aa, Artificial Sequence
  msLacBP6_187C_D220E  (187C, 220E double substitution mutant with signal peptide replaced with M and a GGSHHHHHH at C-terminus)
MATTWKIQSVWDAGTVGYDLFKEWCDGMEEKTGGELKFTCFPAKAVAADNNGLFDAVRNGVLQGMNPFTLYWSGKIPASVFLSSYPAGPDQPHQWDTMFYSLGMLEKTREIYKKFGLFYVGPIQHDANIIHSKQPINSLDDLKGLKMRLPGGMVAEVFAKFGVAAVSLPGSDIFPALEKGTIDAADCVGPAVNWELGFSQVTKYILMGPPGIMSVYQPVELMDLTVNLRAWNALDPKLQQIVEDEVRIYSQKHYLAIQKRNIEAMKKFEAAGTTVTRLSQEDLQEFRRAAIPIWYSWANKDEDAREIFDMQLEYMMNDTVGYITEDDIKGMNGGSHHHHHH

SEQ ID NO: 57 - protein, 341 aa, Artificial Sequence
  msLacBP6_187C_D220L  (187C, 220L double substitution mutant with signal peptide replaced with M and a GGSHHHHHH at C-terminus)
MATTWKIQSVWDAGTVGYDLFKEWCDGMEEKTGGELKFTCFPAKAVAADNNGLFDAVRNGVLQGMNPFTLYWSGKIPASVFLSSYPAGPDQPHQWDTMFYSLGMLEKTREIYKKFGLFYVGPIQHDANIIHSKQPINSLDDLKGLKMRLPGGMVAEVFAKFGVAAVSLPGSDIFPALEKGTIDAADCVGPAVNWELGFSQVTKYILMGPPGIMSVYQPVLLMDLTVNLRAWNALDPKLQQIVEDEVRIYSQKHYLAIQKRNIEAMKKFEAAGTTVTRLSQEDLQEFRRAAIPIWYSWANKDEDAREIFDMQLEYMMNDTVGYITEDDIKGMNGGSHHHHHH

SEQ ID NO: 58 - protein, 341 aa, Artificial Sequence
  msLacBP6_187C_D220N  (187C, 220N double substitution mutant with signal peptide replaced with M and a GGSHHHHHH at C-terminus)
MATTWKIQSVWDAGTVGYDLFKEWCDGMEEKTGGELKFTCFPAKAVAADNNGLFDAVRNGVLQGMNPFTLYWSGKIPASVFLSSYPAGPDQPHQWDTMFYSLGMLEKTREIYKKFGLFYVGPIQHDANIIHSKQPINSLDDLKGLKMRLPGGMVAEVFAKFGVAAVSLPGSDIFPALEKGTIDAADCVGPAVNWELGFSQVTKYILMGPPGIMSVYQPVNLMDLTVNLRAWNALDPKLQQIVEDEVRIYSQKHYLAIQKRNIEAMKKFEAAGTTVTRLSQEDLQEFRRAAIPIWYSWANKDEDAREIFDMQLEYMMNDTVGYITEDDIKGMNGGSHHHHHH

SEQ ID NO: 59 - protein, 341 aa, Artificial Sequence
  msLacBP6_187C_D220Q  (187C, 220Q double substitution mutant with signal peptide replaced with M and a GGSHHHHHH at C-terminus)
MATTWKIQSVWDAGTVGYDLFKEWCDGMEEKTGGELKFTCFPAKAVAADNNGLFDAVRNGVLQGMNPFTLYWSGKIPASVFLSSYPAGPDQPHQWDTMFYSLGMLEKTREIYKKFGLFYVGPIQHDANIIHSKQPINSLDDLKGLKMRLPGGMVAEVFAKFGVAAVSLPGSDIFPALEKGTIDAADCVGPAVNWELGFSQVTKYILMGPPGIMSVYQPVQLMDLTVNLRAWNALDPKLQQIVEDEVRIYSQKHYLAIQKRNIEAMKKFEAAGTTVTRLSQEDLQEFRRAAIPIWYSWANKDEDAREIFDMQLEYMMNDTVGYITEDDIKGMNGGSHHHHHH

SEQ ID NO: 60 - protein, 341 aa, Artificial Sequence
  msLacBP6_187C_D220S  (187C, 220S double substitution mutant with signal peptide replaced with M and a GGSHHHHHH at C-terminus)
MATTWKIQSVWDAGTVGYDLFKEWCDGMEEKTGGELKFTCFPAKAVAADNNGLFDAVRNGVLQGMNPFTLYWSGKIPASVFLSSYPAGPDQPHQWDTMFYSLGMLEKTREIYKKFGLFYVGPIQHDANIIHSKQPINSLDDLKGLKMRLPGGMVAEVFAKFGVAAVSLPGSDIFPALEKGTIDAADCVGPAVNWELGFSQVTKYILMGPPGIMSVYQPVSLMDLTVNLRAWNALDPKLQQIVEDEVRIYSQKHYLAIQKRNIEAMKKFEAAGTTVTRLSQEDLQEFRRAAIPIWYSWANKDEDAREIFDMQLEYMMNDTVGYITEDDIKGMNGGSHHHHHH

SEQ ID NO: 61 - protein, 362 aa, Artificial Sequence
  msLacBP6_187C_bZifC (187C substitution mutant, with bZif fusion, signal peptide replaced with M and a GGSHHHHHH at C-terminus)
MATTWKIQSVWDAGTVGYDLFKEWCDGMEEKTGGELKFTCFPAKAVAADNNGLFDAVRNGVLQGMNPFTLYWSGKIPASVFLSSYPAGPDQPHQWDTMFYSLGMLEKTREIYKKFGLFYVGPIQHDANIIHSKQPINSLDDLKGLKMRLPGGMVAEVFAKFGVAAVSLPGSDIFPALEKGTIDAADCVGPAVNWELGFSQVTKYILMGPPGIMSVYQPVDLMDLTVNLRAWNALDPKLQQIVEDEVRIYSQKHYLAIQKRNIEAMKKFEAAGTTVTRLSQEDLQEFRRAAIPIWYSWANKDEDAREIFDMQLEYMMNDTVGYITEDDIKGMNGGSTGEKPYKCPECGKSFSRSGGSHHHHHH

SEQ ID NO: 62 - protein, 362 aa, Artificial Sequence
  msLacBP6_188C_bZifC (188C substitution mutant, with bZif fusion, signal peptide replaced with M and a GGSHHHHHH at C-terminus)
MATTWKIQSVWDAGTVGYDLFKEWCDGMEEKTGGELKFTCFPAKAVAADNNGLFDAVRNGVLQGMNPFTLYWSGKIPASVFLSSYPAGPDQPHQWDTMFYSLGMLEKTREIYKKFGLFYVGPIQHDANIIHSKQPINSLDDLKGLKMRLPGGMVAEVFAKFGVAAVSLPGSDIFPALEKGTIDAADYCGPAVNWELGFSQVTKYILMGPPGIMSVYQPVDLMDLTVNLRAWNALDPKLQQIVEDEVRIYSQKHYLAIQKRNIEAMKKFEAAGTTVTRLSQEDLQEFRRAAIPIWYSWANKDEDAREIFDMQLEYMMNDTVGYITEDDIKGMNGGSTGEKPYKCPECGKSFSRSGGSHHHHHH

SEQ ID NO: 63 - DNA, 1451 bp, Artificial Sequence
  Exemplary ttLacBP1 expression sequence.
gccagtaagcttcggtcacgcttgggactgccataggctggcccggtgatgccggccacgatgcgtccggcgtagaggatcgagatctcgatcccgcgaaattaatacgactcactatagggagaccacaacggtttccctctagaaataattttgtttaactttaagaaggagatataccatgtttagtcctttagcagtagcacaagctcgtcgctatcgttggcgtattcagacagcatgggacgcagggaccgtggggtactctctttttcaaaagtttaccgagcgcgtaaaagaactcacagacgggcagttagaggtacaaccgttcccggctggtgcggtagtagggacctttgacatgttcgacgccgtcaagacaggtgtattagacgggatgaatcctttcacactctattgggccggtcgtatgccagtcaccgcatttttgagcagttacgcgctgggtctcgatcggccagaccaatgggaaacgtggttctacagtctcggcggtttagatatcgcacgccgtgcgttcgcggagcagggtctcttttacgtagggccagtacaacacgatctcaatattattcattcaaagaagccaatccgccgtttcgaagacttcaagggtgtaaagttacgggtaccgggtggcatgattgctgaagtcttcgcagctgcaggtgcctcaacagtgctcctccctggcggggaagtatatccggccttagagcgtggtgtcatcgacgcagccgatttcgtaggtccagccgttaattacaacttaggtttccaccaggtagccaaatacatcatcatgggtccaccagaaacaccggcaattcatcaaccagtagacctcatggactttacgatcaatctgaatcgttggcgtagtttgccaaaaccattacaagaacgcttcattgcagctgtccatgagtattcctggatccattacgctggcattcaaaaggcgaatctggaagcctggccaaaataccggcaagcaggtgtcgaagtcatccggttatccaatgaagacgtgcgtaaattccgtcgtctcgccattcctatctggtttaagtgggcaaaaatggacaaatatagccgtgaggcattcgccagtcaattggaatacatgaagggcattgggtacgtaaccgacgaggaattaaagggtttgtccttaggtggttcacatcatcatcatcatcattaatgaaagggcgatatccagcacactggcggccgttactagtggatccggctgctaacaaagcccgaaaggaagctgagttggctgctgccaccgctgagcaataactagcataaccccttggggcctctaaacgggtcttgaggggttttttgctgaaaggaggaactatatccggagcgactcccacggcacgttggcaagctcggaattcggcgtaatc

SEQ ID NO: 64 - DNA, 1451 bp, Artificial Sequence
  Exemplary tsLacBP2 expression sequence.
gccagtaagcttcggtcacgcttgggactgccataggctggcccggtgatgccggccacgatgcgtccggcgtagaggatcgagatctcgatcccgcgaaattaatacgactcactatagggagaccacaacggtttccctctagaaataattttgtttaactttaagaaggagatataccatgtttagtccattagcagtagcacaagcaccacgttttcgttggcgtatccaatctgcctgggacgcagggacagtgggctattccctttttcaaaaatttgccgaacgggtcaaggaactcacggacggtcaaattgaaatccagacattcccagcaggcgcggtcgttggtactttcgatatgtttgacgcagtaaaaaccggggtcctcgatgggatgcacccgtttaccctctactgggccggccggatgccagtcactgcttttttgtcatcatatccacttggcctcgaccggcctgatcaatgggagacgtggtattacggcctcggtggtctggaattagcacgtaaagcatatgaagaacaaggcctcttttttgtcggcccggttcaacacgattacaacttaattcattccaaaaagccaatcaaatcattcgaggattttaagggtgtcaaactccgcgtcccaggcggcatgattgccgagattttcgccgcagcaggggccgcaacagtactcctcccaggcggggaagtctatccggcccttgagcgtggtgtcatcgacgcggccgacttcgtaggtccagccgtaaactacaatttaggttttcatcaagtcaccaaatacatcatcatgggcccgcctgaaacaccggccattcaccagccagtcgacttagccgacattaccattaatatcaatcgctggcgggcgcttccacgtaacctgcaagaacgctttgaggctgccgtgcacgagtggtcctggattcactatgccggtattcaaaaggcgaaccttgagacctggccgaagtacaaagccgccggcgtgcaagtgattcgcttatccaccgtagacgtccgtaaatttcgccgtgtcgcgatcccaatttggttcaagtgggcgaaacaggacaaatatacacgcgaggcattcgcaagtcaattggagtatatgaaagcattaggttatgtaacagacgcagacatccgggggctgagcttaggtggttctcatcatcatcatcatcattaatgaaagggcgatatccagcacactggcggccgttactagtggatccggctgctaacaaagcccgaaaggaagctgagttggctgctgccaccgctgagcaataactagcataaccccttggggcctctaaacgggtcttgaggggttttttgctgaaaggaggaactatatccggagcgactcccacggcacgttggcaagctcggaattcggcgtaatc

SEQ ID NO: 65 - DNA, 1511 bp, Artificial Sequence
  Exemplary toLacBP3 expression sequence.
gccagtaagcttcggtcacgcttgggactgccataggctggcccggtgatgccggccacgatgcgtccggcgtagaggatcgagatctcgatcccgcgaaattaatacgactcactatagggagaccacaacggtttccctctagaaataattttgtttaactttaagaaggagatataccatgaaatcaacacggcgtcaatttttaaaaaaagcagcaatcggtgtggccgcctcctcagcattttcacctctcgcaatcgcgcaggctccacggttccgttggcgtatccaatcggcatgggacgcaggcacagtaggttacacgttatttcaacgcttcgccgaacgcgtcaaagagcttacagacggccagattgaaattcagccttttccggcaggcgcagtcgtaggcaccttcgatatgttcgacgcggtgaaaacaggggtcctcgatgggatgcacccatttaccctgtactgggctggccgtatgcctgtcaccgcattcttatcatcctacccgcttggcttagatcgcccagatcaatgggaaacctggtactacggcttagggggcttggagttagcccgtaaagcatatgaggagcagggtttggcatatattggcccagtacaacacgattataacctcatccattcaaagaaacctattaagtcgttcgaagagttcaaaggcgtcaagttacgcgtgccaggtgggatgatcgctgaaatcttcgcagcagcaggtgcggctactgtcttattaccagggggggaagtctacccggctctcgagcgtggcgtcattgatgcagctgatttcgtaggcccagctgtcaattacaatttaggctttcatcaagtaacaaagtatatcattatgggcccgccagaaacaccggccattcaccaaccagtagacctcgcggatatcaccttgaacttaaatcgttggcgggcagtacctaagaatttgcaagagcgcttcgaagccgctgtacacgaatggtcatgggtccattacgcaggcatccaaaaagccaacctcgaagcctggccaaaatatcgggctgcaggtgtgcagatcatccgcttaagtacagttgacgtccgcaagtttcgtcgtgtggcaattccgatttggttcaaatgggcaaagcaagacaagtatgcaaaagaagcctttcaatcacagctggaatacatgaaggcgttagggtatgttaccgacgtcgacctgcggggtttgtccttaggtggttcacatcatcatcatcatcattaatgaaagggcgatatccagcacactggcggccgttactagtggatccggctgctaacaaagcccgaaaggaagctgagttggctgctgccaccgctgagcaataactagcataaccccttggggcctctaaacgggtcttgaggggttttttgctgaaaggaggaactatatccggagcgactcccacggcacgttggcaagctcggaattcggcgtaatc

SEQ ID NO: 66 - DNA, 1442 bp, Artificial Sequence
  Exemplary tsLacBP4 expression sequence.
gccagtaagcttcggtcacgcttgggactgccataggctggcccggtgatgccggccacgatgcgtccggcgtagaggatcgagatctcgatcccgcgaaattaatacgactcactatagggagaccacaacggtttccctctagaaataattttgtttaactttaagaaggagatataccatgacagcacgtggtgttcgttggcgtatgcaatcagcatggcaaccaggcacaatcggttatcgtacattcgaaacttgggcacgttccattcaagagctcaccagtggtgaattgtcgatcgaaccttttccggccggggcagtagccggtaccttcgaaatggcagacgcggtccggtctggggtcctcgacggcatgaattggttcactgtctattggccggggaaaatgccagcaggtgtctttatgtcggcgtaccctatggcgctctccctgccacaccactgggatatgatgttcgattcttttgggggccgtcagatcgtcgacgagctctacgaccgtcaggggcttgtatttctcggccatgtacaacacgatctcaatttaattcactcaaaagttcctttgcgttccttcgacgactttcggggtaagcgtattcgttttccaggtggtattatcgcagaaacatttgccaaggtcggcgtacgtacaacattattaccggggggtgacgtatatccggccttagagcgtggtaccattgacgcagcagactttgtaggcccagcggtaaactacgatttaggttttcatcaggtggccgattatatcatcatgggccctccaagtaccccagcgttacaccaaccagttgatctcatggacatctctgtaaacaagcgtagctggtcgcgtatctcggagcacacccagaaattaatgtataaattcgtcaaagcatattccgcagagcactttgcagccatccaaaaagccaaccatgaggcatggccgaaatacaaggaggccggtgtcgaagtcatccacttaagtgaagaggatgcagcacgtttccgggaggcagcaatcccgctctggttcgaatgggcaaacaaagaccgtgatgcggcccggctctttaaggttcatttagaagtcatgcaagacccatcggtagcggtcatcaccccagatgacattaaagattacaaattgaactttggcggttctcatcatcatcatcatcattaatgaaagggcgatatccagcacactggcggccgttactagtggatccggctgctaacaaagcccgaaaggaagctgagttggctgctgccaccgctgagcaataactagcataaccccttggggcctctaaacgggtcttgaggggttttttgctgaaaggaggaactatatccggagcgactcccacggcacgttggcaagctcggaattcggcgtaatc

SEQ ID NO: 67 - DNA, 1442 bp, Artificial Sequence
  Exemplary rdLacBP5 expression sequence.
gccagtaagcttcggtcacgcttgggactgccataggctggcccggtgatgccggccacgatgcgtccggcgtagaggatcgagatctcgatcccgcgaaattaatacgactcactatagggagaccacaacggtttccctctagaaataattttgtttaactttaagaaggagatataccatggcagctggtgaaggtacaacttggaaaattcagacaagtcataccggtggtattggcctcgcgacttttaaagactgggcgtcctctatcgaggagaagacgggtggtgagttagcctttacagcttttggtgccaatgatgtggtaggtgactttcaactttacgacgcagtcaaaaacggtgttttagatgcggtcaacccattcacaatttatgcacaaggtatcatcccggctgcaacatttctgacttcatacccactcggtctccgcaatccgcacgaatgggacgtcttcttttacagccttggcggcctcgaaattgcccgtgaactctacgccgcacaaggtatgaaattcgtcgggcctgtccatcatggtccaaatatcattcattcgaaggtgcctattcgttccatcgatgacttcgcgggtctcaaaatgcgtatgccaggcggcatggtcgcagaagtcttcagtgaaatcggtgccgagacaaccgtcttacctggtagcgagattttcccggcgcttgaaaaaggtacaatcgacgccgctgacttcgttggcccagcagtaaattatgcgttaggcttcagccaggtcaccaactatatttccatgggtccagccggtttcatgtccttgtaccaaccagtagatttaatggatattacggtaggccaaaccgcatgggacgcactctcaccgcagatgcaacagtttgtagagatggaaacccacgtatacagcgacatgcatcacgccgccattcaaaaagcagaccaagaggcatgggctaaattcgaggccgacggtactgaggttacccgtttgtcccaagatgatgtagaattaatgaccgaagtcgccgttccaatctggttcgactatgcaaaccgtgataaggacgcagcacgggtcttcaaaatccaattagactacatgatgtcaggcagtctcgggtatgtgacaccagaacaaattgaaggcttgaccttgaatttaggtggttcacatcatcatcatcatcattaatgaaagggcgatatccagcacactggcggccgttactagtggatccggctgctaacaaagcccgaaaggaagctgagttggctgctgccaccgctgagcaataactagcataaccccttggggcctctaaacgggtcttgaggggttttttgctgaaaggaggaactatatccggagcgactcccacggcacgttggcaagctcggaattcggcgtaatc

SEQ ID NO: 68 - DNA, 1400 bp, Artificial Sequence
  Exemplary msLacBP6 expression sequence.
cggtcacgcttgggactgccataggctggcccggtgatgccggccacgatgcgtccggcgtagaggatcgagatctcgatcccgcgaaattaatacgactcactatagggagaccacaacggtttccctctagaaataattttgtttaactttaagaaggagatataccatggcaacaacttggaaaattcaaagtgtatgggatgcagggacggtgggctatgacctcttcaaggagtggtgcgacggtatggaagaaaagacgggcggtgaactcaaattcacgtgcttcccagccaaagccgtcgccgcagataataatggtctttttgatgcagtacggaatggcgtcttgcaaggtatgaatcctttcaccctctactggtcaggtaagattccggcctccgtatttctctcgtcgtacccagccggtccagatcaaccacatcaatgggatacaatgttctacagccttggtatgttagaaaaaacacgtgaaatttacaaaaagttcggcctcttctacgtcggcccaattcagcacgacgcaaacattatccacagtaaacagccgattaattccctggacgaccttaagggtctcaaaatgcgcttacctggcgggatggtagcggaagtctttgcaaagtttggcgtcgcagcggtcagtctcccaggcagcgacatctttccagccttagaaaaaggcacaatcgacgctgctgattacgtgggtccggctgtaaactgggagctcggcttcagccaagtaacaaagtacatcttaatgggtccaccaggcatcatgtcagtctaccaaccggtcgaccttatggacctcactgtcaatctgcgggcctggaacgcattagatccaaagttacagcaaatcgttgaagatgaagtacgcatctactctcagaagcattacctcgcaattcagaaacggaatattgaagctatgaagaagttcgaggccgctggtacaaccgtaacccgtctgtcacaagaggacctccaggagtttcgtcgtgcagctatcccaatttggtattcatgggcaaacaaagatgaagacgcacgggagattttcgacatgcaattagagtacatgatgaacgacactgtaggttacatcactgaagatgacattaagggcatgaatggcggttcacatcatcatcatcatcattaatgaaagggcgatatccagcacactggcggccgttactagtggatccggctgctaacaaagcccgaaaggaagctgagttggctgctgccaccgctgagcaataactagcataaccccttggggcctctaaacgggtcttgaggggttttttgctgaaaggaggaactatatccggagcgactcccacggcacgttggcaagctcg

SEQ ID NO: 69 - DNA, 1406 bp, Artificial Sequence
  Exemplary tsLacBP7 expression sequence.
cggtcacgcttgggactgccataggctggcccggtgatgccggccacgatgcgtccggcgtagaggatcgagatctcgatcccgcgaaattaatacgactcactatagggagaccacaacggtttccctctagaaataattttgtttaactttaagaaggagatataccatgcaagcaccacgttttcgttggcgtattcaaagtgcatgggatgcaggaacagtgggttacaccctctttcagcgctttgcagaacgcgtcaaagagctgaccgatggacagatcgagatccagacctttccagcgggtgcagtcgtgggtaccttcgacatgttcgacgcagtcaaaaccggagtgctggatggcatgcatccctttaccctctattgggcaggtcgaatgccggttaccgcctttctcagcagctacccgttaggcctggatcgaccagatcagtgggaaacgtggtactacgcacttggcggtctggatctggcgagacgtgcattcgaggaacagggtctgttctacgttggtccagtgcagcatgactacaacctgatccacagcaaaaagccgatcaagtccttcgaggacttcaaaggcgtgaagctgagagtgcctggtggcatgatagcagacgtcttctcagcagctggagcagcaacagtcctcttgcctggtggtgaggtctatccggctctggaacgtggtgtgatcgatgcagcagacttcgtgggtcctgcagtgaactacaaccttggcttccatcaggtgaccaagtacatcatcatgggtcctccagaaacccctgcgatccatcagccagtggatctggcagacatcaccctgaacctcagccgttggcgtgcagtgcccaaaaacctgcaggaacgattcgaagcagcggttcacgaatggagctggatccactatgccggtatccagaaagccaacctggagacctggccgaagtacaaagcggcaggtgtgcagatcatcaggctgactaccgtggatgtgcgcaagtttcgtcgtgttgcgattccgatctggttcaaatgggcgaaacaggacaagtatgcccgtgaagcctttgcaagccagctggagtacatgaaagcactgggctatgtgacagatgcagatgttcgtggtttaagcttaggcggcagccatcatcatcatcatcattaataatgaaagggcgatatccagcacactggcggccgttactagtggatccggctgctaacaaagcccgaaaggaagctgagttggctgctgccaccgctgagcaataactagcataaccccttggggcctctaaacgggtcttgaggggttttttgctgaaaggaggaactatatccggagcgactcccacggcacgttggcaagctcg

SEQ ID NO: 70 - DNA, 1406 bp, Artificial Sequence
  Exemplary maLacBP8 expression sequence.
cggtcacgcttgggactgccataggctggcccggtgatgccggccacgatgcgtccggcgtagaggatcgagatctcgatcccgcgaaattaatacgactcactatagggagaccacaacggtttccctctagaaataattttgtttaactttaagaaggagatataccatgcaagcagcaactacttggaaaattcaaagtacctgggatgctggtacggttggctacaccctcttcgaagagtgggcgaagagcatcgaagccaaatccggtggtgaactgaagttccaggcgtttccggcaaaagccgttgctgctgacaacaacgcgctctttgacgctgttcgcaacggtgtgcttcagggcatgaacccgttcaccctgtactgggcgggcaaaatccctgcctctgtgttcctgtcgagctacccagcaggtccggatcaaccccatcagtgggataccatgttctactcgatgggtatgctggagaaaacccgcgaaatctacaagaaatttggcctgttctacgttggtccgatccagcatgatgcgaacatcatccacagcaaacagccagtcaactctctggacgacctgaaagggatgaagatccgtgtacctggtggcatggttgccgaagtcttccagcagtttggcgtttccaccgtcagtctgccgggtagcgacatcttcccggcattggagaaaggcacgattgacgctgcagacttcgtaggtccagcagtcaactacgaactgggctttagccaggttacggactacatcatcttcggaccacctggcgtcatgagcatctatcaaccggtggacctgatggatctgaccgtcagtctgcgtgcttggaactcgatctcaccagagctgcagcagctggttgaggatgaagtgcgcatctactcgcagaaacactatctggcgattcaggctcgcaacatcgaagcgatggagaaattcaaagccgatggtgacacggtaacccgtctgagccaggaagacctggaaacctggcgtaaggctgcaatcccgatctggttcaactgggcgaacaagaacgatgatgctcgtgcgatcctggatatccagctgaaatacatgatgaacgacactgtgggctacattactgaagaagatattaaaggatttggcggcagccatcatcatcatcatcattaatgataaaagggcgatatccagcacactggcggccgttactagtggatccggctgctaacaaagcccgaaaggaagctgagttggctgctgccaccgctgagcaataactagcataaccccttggggcctctaaacgggtcttgaggggttttttgctgaaaggaggaactatatccggagcgactcccacggcacgttggcaagctcg

SEQ ID NO: 71 - DNA, 1439 bp, Artificial Sequence
  Exemplary adLacBP9 expression sequence.
cggtcacgcttgggactgccataggctggcccggtgatgccggccacgatgcgtccggcgtagaggatcgagatctcgatcccgcgaaattaatacgactcactatagggagaccacaacggtttccctctagaaataattttgtttaactttaagaaggagatataccatgcaagcaccaattactctgagatttcagagtacttggccgcagaaagacatcttccacgagtttgccctggattacgccaaaaaggtcaacgagatgagcggtggacgtctgaagatcgaggttctggcagcaggcagtgtggtgaaggcgttcgatctcctggatgcagtgagcaagggtacgctggatggaggtcatggcgtagtcgcctactggtacggcaagaacaccgcattagcgctgtggggctctggacctgcattcggcatggacccaaacatggtgcttgcatggcaccattacggcggaggtcgtcagctcctggaagagatctaccgaagcctcaacctggatgtcgtcagcctcatgtacggaccaatgccgactcagccgttaggctggttcaagcagaaacccattgcgaaacctgacgacatgaaagggctgaagttccgtacggtaggtctgagcatcgacatcttcaacggactgggtgctgcagtgaacgcgttaccaggtgccgaaatcgttccggctatggatcgaggtctgctcgatgcggcagagttcaacaacgcttcttccgatcgtgtgctagggtttccggatgtctcgaagatcgcgatgctgcaatcgttccatcaggcgtcagagcagttcgagatcctgttcaacggcaagcgtttccaggcgttaccggctgatctgaagagcatcatctccattgctgcgcaagctgcaagcgccgacatgtcctggaaggccatcgatcgctactctagcgactacttcgagatgcgtgacaagcagggcgtgaagttctacagcaccagaccggaaatcctgaaacggcaactggagatctgggaccaggtgatggagaagcgtgcagccgaaaacccgacgttcaaaaaggtcctggagagccaacgcaggtttgcacagcgtgctgcgagatggcagaacgacaccaacgtggacttcaagatggcctacaaccacttctttggtggtaagaaaaaagctactggcggcagccatcatcatcatcatcattaataatgaaagggcgatatccagcacactggcggccgttactagtggatccggctgctaacaaagcccgaaaggaagctgagttggctgctgccaccgctgagcaataactagcataaccccttggggcctctaaacgggtcttgaggggttttttgctgaaaggaggaactatatccggagcgactcccacggcacgttggcaagctcg

SEQ ID NO: 72 - DNA, 1355 bp, Artificial Sequence
  Exemplary pgLacBP10 expression sequence.
cggtcacgcttgggactgccataggctggcccggtgatgccggccacgatgcgtccggcgtagaggatcgagatctcgatcccgcgaaattaatacgactcactatagggagaccacaacggtttccctctagaaataattttgtttaactttaagaaggagatataccatgcaagaagcagttgaatggagaatgcaagcattgtgggatgcaggtacgaccccattcgaattcgaaaagaagttcgtggaacgtgtaggcgagttgacggaaggtcgcttcaagatcacgctgtacagcgcaggtcagatagtgccggcaaaccaggccttcgatgctgtgcgttctggtgccttcgagatgatgaaaaccttcgatggctatgaggcaggcaaaatcccggcattcgccttcacctcgaccattccgttcggtttcccgcagtctgaccagtacgaggcatggttctacgaactgggtggtctggatcttgctcgcgaagcttacgccaaaggtggcctgttctacatcgcaccgaccgtctatggcgaagaacccatgcacagcaccgtgaagatcgaatccatcgcggatatggcggggaagaaaggccgttttgtcggtttggcatctgcggtgatggcagatctcggtgtagcggtgtcgccgttagcgactgccgaagtgtacactgcgctcgaaaaaggcctgatcgactttgcggatcgtggtgatctgacagccaactacgaagcaggacttggcgaagtggcgaaattcatcatccttccgggtgtgcatcaaccgaccactgcaaccagctatgtcgcgaatcaggcagcgtaccagaagcttccggatggcttcaaagcggcgttagcggttgctgcacgtgagatctccggttcactgcgtcagcacatcctggttcaggacatggaagtgctcaccaagtacaaggatcagggtgtggaagtggtacgtctcgatgcagcggatattgctgcggcaagagcgaaagcggtcgaatcctgggaaaaggcgaccaaaggggatgaactggcgaccagagtgctgaagggacaggtggattttatgacttctttaggtttactgggcggcagccatcatcatcatcatcattaataatgaaagggcgatatccagcacactggcggccgttactagtggatccggctgctaacaaagcccgaaaggaagctgagttggctgctgccaccgctgagcaataactagcataaccccttggggcctctaaacgggtcttgaggggttttttgctgaaaggaggaactatatccggagcgactcccacggcacgttggcaagctcg

SEQ ID NO: 73 - DNA, 1415 bp, Artificial Sequence
  Exemplary psLacBP11 expression sequence.
cggtcacgcttgggactgccataggctggcccggtgatgccggccacgatgcgtccggcgtagaggatcgagatctcgatcccgcgaaattaatacgactcactatagggagaccacaacggtttccctctagaaataattttgtttaactttaagaaggagatataccatgcaacaagcagcaggtgaaccagcaaaaacctatcactggaagatggtgaccgcttggccgaagaactatccgggtttaggcaccagtgcggaacgactggcagaacgtgtgaacgcgatgagtggtggacgtctgaccatcaaggtgtatgcagcaggagaactggttccagctctggaagtgttcgatgcagtctctcgtggtaccgcagaactgggtcatggagcaagctactactggaaaggcaaggttccgactgcgcagttcttcaccagtgtaccgtttggtctgtcaaccagcgagatgaacgcatggctgagcaaaggtggtggacaggcgttctgggacgaagcctacgctcctttcggcgtgaaaccgcttgtgatcggcaataccggcatgcagatgggtggatggtacaacaaagagatcaacagcctgactgacctcaaaggcctgaaaatccgcatgccaggtctgggtggtgaagtgctaagcagactgggtgcaaccaccgtgaaccttccaggtggtgaagtctttaccgcactgcagacaggagcgatcgatgcaaccgattgggtgagtccctacaacgatctggcctttggtctgcacaaagcagcacgctactactactacccgggttggcaggaaccacaggctgtactggaactgctgatcaaccagaaggcgttcgatagcttaccggcagatctgcaggcgatcgtgaccgaagcaagcctggcagcaagccgcgatatgcatgacgattacgtctacaacaacgctctggctctggaacagctcaaacagcagggaaccgaactgaagcgctttccggacgaagtgctggcagcaatgcgcgaacagtctgacctgatcctcggtgaactggctgcacagagcgaactgaacggtcgtatctgggcaagcatgaaggcctttcaggctcaggtcgaaccgatgcacgagattagcgaaaaagaattgtataattggagaggcggcagccatcatcatcatcatcattaataatgaaagggcgatatccagcacactggcggccgttactagtggatccggctgctaacaaagcccgaaaggaagctgagttggctgctgccaccgctgagcaataactagcataaccccttggggcctctaaacgggtcttgaggggttttttgctgaaaggaggaactatatccggagcgactcccacggcacgttggcaagctcg

SEQ ID NO: 74 - DNA, 1415 bp, Artificial Sequence
  Exemplary fsLacBP13 expression sequence.
cggtcacgcttgggactgccataggctggcccggtgatgccggccacgatgcgtccggcgtagaggatcgagatctcgatcccgcgaaattaatacgactcactatagggagaccacaacggtttccctctagaaataattttgtttaactttaagaaggagatataccatggaaaaaaaaattcgttggaaattagcaatgacttggggtccgaccttgcatccgttgtccgacacagcagagcatatggcggaaatcgtgaaggagttgagcgatggcaacttcgtgatcaacatcgatgcgtcgaacgtgcacaaagcgccgtttggcatcttcgatatggtgaaactcggtcagtacgagatgggccatactgcgagctactactacaaaggcaaaaacatcgcgtttttaccgctgacgaccatgcctttcggtatgaccgcaccggaacagtatgcgtggttctactatggtggcggtctggagctgatgcaggaagcgtacaccaagcatggcatgctggcgtttcctggtggtaacaccggtaaccagatgggaggttggttcaccaaggagatcaacagcctggatgacctcaagggtctcaagatgaggatcccaggctttgcgggccagatcatgtccaaactgggtgtgaccgtgaccaacatccctccaggtgagctgtacaccgcactggaacgtggtaccgtggatgcggtggaatggaccggtcctggtatggacatcaacatgggattccacaagatcgcgaaatactactataccggttggcatgaaccgggatccgaagtggagttcctgatcaacgaaaaggaatacaacaaactgccggaaaaatacaaaaagatcctgaaaatcgccatgaaaaccgcagcgtacgacatgtacatccagtcgtacgagatgaacgctgaagcttggcagcagatgaaagagaaatacccggatatcaaggtcaaggtttttccggaagaagtgctgaaagagatgaagaccgcgtacgacaaccttgtggcgagctacgagaaagaaagcccgatgttcaagaaaatcatggagagcaaacgtgcgtatctggacaaggttcgagactggacccacatatcggactacctctacctgaaaagtacttctgaaagtaatctgaatggcggcagccatcatcatcatcatcattaatgataaaagggcgatatccagcacactggcggccgttactagtggatccggctgctaacaaagcccgaaaggaagctgagttggctgctgccaccgctgagcaataactagcataaccccttggggcctctaaacgggtcttgaggggttttttgctgaaaggaggaactatatccggagcgactcccacggcacgttggcaagctcg

SEQ ID NO: 75 - DNA, 1400 bp, Artificial Sequence
  Exemplary taLacBP14 expression sequence.
cggtcacgcttgggactgccataggctggcccggtgatgccggccacgatgcgtccggcgtagaggatcgagatctcgatcccgcgaaattaatacgactcactatagggagaccacaacggtttccctctagaaataattttgtttaactttaagaaggagatataccatggaagaatataaatttaaaatggcaactttttacctgaaaggtgatagcgcctttgacgtgatcgaccactttcgccaactggtctggaagaaaaccggtggtaaggtacgcatcgatgcgttccaagctggggaactgggctttccagtgaccgagatcctggaagcgaccagtcgtggtgtggtggagatgagcatcttctacccgaactacaaagcggcacaggatccggtgatggccttagcgggaggacgtccgggtccaatgttcgacctgcgtgatcagaaagcccaagtggatgcgaccaaagatctcctggaaaggtccttcggtcgtttcggagttcgctacattgcgcctatggtgtacggtgaaccggagatcctggtctcgagacgtccgatgagtagcctcaaagacctgaaagggcgtatcttccgtgcgagtggtatggcagcggagttctacaccgcaattggcgcacaagcgatgatgcttccagcaggtgagctctaccaggcactgcagttaggcaccatcgatggtctggagtggaccgactataccgcgaactacaagcttggcttccacgaagtggcgaagaacgtgctggaaccgacgaaaggtgtgaacctccattcggaagctaccgttcatgcgttcctggttgtgaacccgaaagtctgggagaaactgccgaaggaacaccagaaagcgatccaggaagcggcggacgaagcgtacaaatggggtgcggatcaccttgcgaaactgaacaaaacctacaaggacaaatggatcaaagcgggtgcgaaggtgacccaactgccgaaagaagaccaggacaaagtgatcgaagtgtcggcaaagatcctgtctggctatagcgcgaagagtccggatgcgaaagagtacgcgcgtcgtctagtggagctgtggaagaaactgggctacaccaaatggtctgatgcattagcaaaacagattaaaggcggcagccatcatcatcatcatcattaataatgaaagggcgatatccagcacactggcggccgttactagtggatccggctgctaacaaagcccgaaaggaagctgagttggctgctgccaccgctgagcaataactagcataaccccttggggcctctaaacgggtcttgaggggttttttgctgaaaggaggaactatatccggagcgactcccacggcacgttggcaagctcg

SEQ ID NO: 76 - DNA, 1400 bp, Artificial Sequence
  Exemplary msLacBP6.10C expression sequence.
cggtcacgcttgggactgccataggctggcccggtgatgccggccacgatgcgtccggcgtagaggatcgagatctcgatcccgcgaaattaatacgactcactatagggagaccacaacggtttccctctagaaataattttgtttaactttaagaaggagatataccatggcaacaacttggaaaattcaaagttgttgggatgcagggacggtgggctatgacctcttcaaggagtggagcgacggtatggaagaaaagacgggcggtgaactcaaattcacggcgttcccagccaaagccgtcgccgcagataataatggtctttttgatgcagtacggaatggcgtcttgcaaggtatgaatcctttcaccctctactggtcaggtaagattccggcctccgtatttctctcgtcgtacccagccggtccagatcaaccacatcaatgggatacaatgttctacagccttggtatgttagaaaaaacacgtgaaatttacaaaaagttcggcctcttctacgtcggcccaattcagcacgacgcaaacattatccacagtaaacagccgattaattccctggacgaccttaagggtctcaaaatgcgcttacctggcgggatggtagcggaagtctttgcaaagtttggcgtcgcagcggtcagtctcccaggcagcgacatctttccagccttagaaaaaggcacaatcgacgctgctgattacgtgggtccggctgtaaactgggagctcggcttcagccaagtaacaaagtacatcttaatgggtccaccaggcatcatgtcagtctaccaaccggtcgaccttatggacctcactgtcaatctgcgggcctggaacgcattagatccaaagttacagcaaatcgttgaagatgaagtacgcatctactctcagaagcattacctcgcaattcagaaacggaatattgaagctatgaagaagttcgaggccgctggtacaaccgtaacccgtctgtcacaagaggacctccaggagtttcgtcgtgcagctatcccaatttggtattcatgggcaaacaaagatgaagacgcacgggagattttcgacatgcaattagagtacatgatgaacgacactgtaggttacatcactgaagatgacattaagggcatgaatggcggttcacatcatcatcatcatcattaatgaaagggcgatatccagcacactggcggccgttactagtggatccggctgctaacaaagcccgaaaggaagctgagttggctgctgccaccgctgagcaataactagcataaccccttggggcctctaaacgggtcttgaggggttttttgctgaaaggaggaactatatccggagcgactcccacggcacgttggcaagctcg

SEQ ID NO: 77 - DNA, 1400 bp, Artificial Sequence
  Exemplary msLacBP6.12C expression sequence.
cggtcacgcttgggactgccataggctggcccggtgatgccggccacgatgcgtccggcgtagaggatcgagatctcgatcccgcgaaattaatacgactcactatagggagaccacaacggtttccctctagaaataattttgtttaactttaagaaggagatataccatggcaacaacttggaaaattcaaagtgtatggtgtgcagggacggtgggctatgacctcttcaaggagtggagcgacggtatggaagaaaagacgggcggtgaactcaaattcacggcgttcccagccaaagccgtcgccgcagataataatggtctttttgatgcagtacggaatggcgtcttgcaaggtatgaatcctttcaccctctactggtcaggtaagattccggcctccgtatttctctcgtcgtacccagccggtccagatcaaccacatcaatgggatacaatgttctacagccttggtatgttagaaaaaacacgtgaaatttacaaaaagttcggcctcttctacgtcggcccaattcagcacgacgcaaacattatccacagtaaacagccgattaattccctggacgaccttaagggtctcaaaatgcgcttacctggcgggatggtagcggaagtctttgcaaagtttggcgtcgcagcggtcagtctcccaggcagcgacatctttccagccttagaaaaaggcacaatcgacgctgctgattacgtgggtccggctgtaaactgggagctcggcttcagccaagtaacaaagtacatcttaatgggtccaccaggcatcatgtcagtctaccaaccggtcgaccttatggacctcactgtcaatctgcgggcctggaacgcattagatccaaagttacagcaaatcgttgaagatgaagtacgcatctactctcagaagcattacctcgcaattcagaaacggaatattgaagctatgaagaagttcgaggccgctggtacaaccgtaacccgtctgtcacaagaggacctccaggagtttcgtcgtgcagctatcccaatttggtattcatgggcaaacaaagatgaagacgcacgggagattttcgacatgcaattagagtacatgatgaacgacactgtaggttacatcactgaagatgacattaagggcatgaatggcggttcacatcatcatcatcatcattaatgaaagggcgatatccagcacactggcggccgttactagtggatccggctgctaacaaagcccgaaaggaagctgagttggctgctgccaccgctgagcaataactagcataaccccttggggcctctaaacgggtcttgaggggttttttgctgaaaggaggaactatatccggagcgactcccacggcacgttggcaagctcg

SEQ ID NO: 78 - DNA, 1400 bp, Artificial Sequence
  Exemplary msLacBP6.43C expression sequence.
cggtcacgcttgggactgccataggctggcccggtgatgccggccacgatgcgtccggcgtagaggatcgagatctcgatcccgcgaaattaatacgactcactatagggagaccacaacggtttccctctagaaataattttgtttaactttaagaaggagatataccatggcaacaacttggaaaattcaaagtgtatgggatgcagggacggtgggctatgacctcttcaaggagtggagcgacggtatggaagaaaagacgggcggtgaactcaaattcacggcgttcccatgtaaagccgtcgccgcagataataatggtctttttgatgcagtacggaatggcgtcttgcaaggtatgaatcctttcaccctctactggtcaggtaagattccggcctccgtatttctctcgtcgtacccagccggtccagatcaaccacatcaatgggatacaatgttctacagccttggtatgttagaaaaaacacgtgaaatttacaaaaagttcggcctcttctacgtcggcccaattcagcacgacgcaaacattatccacagtaaacagccgattaattccctggacgaccttaagggtctcaaaatgcgcttacctggcgggatggtagcggaagtctttgcaaagtttggcgtcgcagcggtcagtctcccaggcagcgacatctttccagccttagaaaaaggcacaatcgacgctgctgattacgtgggtccggctgtaaactgggagctcggcttcagccaagtaacaaagtacatcttaatgggtccaccaggcatcatgtcagtctaccaaccggtcgaccttatggacctcactgtcaatctgcgggcctggaacgcattagatccaaagttacagcaaatcgttgaagatgaagtacgcatctactctcagaagcattacctcgcaattcagaaacggaatattgaagctatgaagaagttcgaggccgctggtacaaccgtaacccgtctgtcacaagaggacctccaggagtttcgtcgtgcagctatcccaatttggtattcatgggcaaacaaagatgaagacgcacgggagattttcgacatgcaattagagtacatgatgaacgacactgtaggttacatcactgaagatgacattaagggcatgaatggcggttcacatcatcatcatcatcattaatgaaagggcgatatccagcacactggcggccgttactagtggatccggctgctaacaaagcccgaaaggaagctgagttggctgctgccaccgctgagcaataactagcataaccccttggggcctctaaacgggtcttgaggggttttttgctgaaaggaggaactatatccggagcgactcccacggcacgttggcaagctcg

SEQ ID NO: 79 - DNA, 1400 bp, Artificial Sequence
  Exemplary msLacBP6.49C expression sequence.
cggtcacgcttgggactgccataggctggcccggtgatgccggccacgatgcgtccggcgtagaggatcgagatctcgatcccgcgaaattaatacgactcactatagggagaccacaacggtttccctctagaaataattttgtttaactttaagaaggagatataccatggcaacaacttggaaaattcaaagtgtatgggatgcagggacggtgggctatgacctcttcaaggagtggagcgacggtatggaagaaaagacgggcggtgaactcaaattcacggcgttcccagccaaagccgtcgccgcatgtaataatggtctttttgatgcagtacggaatggcgtcttgcaaggtatgaatcctttcaccctctactggtcaggtaagattccggcctccgtatttctctcgtcgtacccagccggtccagatcaaccacatcaatgggatacaatgttctacagccttggtatgttagaaaaaacacgtgaaatttacaaaaagttcggcctcttctacgtcggcccaattcagcacgacgcaaacattatccacagtaaacagccgattaattccctggacgaccttaagggtctcaaaatgcgcttacctggcgggatggtagcggaagtctttgcaaagtttggcgtcgcagcggtcagtctcccaggcagcgacatctttccagccttagaaaaaggcacaatcgacgctgctgattacgtgggtccggctgtaaactgggagctcggcttcagccaagtaacaaagtacatcttaatgggtccaccaggcatcatgtcagtctaccaaccggtcgaccttatggacctcactgtcaatctgcgggcctggaacgcattagatccaaagttacagcaaatcgttgaagatgaagtacgcatctactctcagaagcattacctcgcaattcagaaacggaatattgaagctatgaagaagttcgaggccgctggtacaaccgtaacccgtctgtcacaagaggacctccaggagtttcgtcgtgcagctatcccaatttggtattcatgggcaaacaaagatgaagacgcacgggagattttcgacatgcaattagagtacatgatgaacgacactgtaggttacatcactgaagatgacattaagggcatgaatggcggttcacatcatcatcatcatcattaatgaaagggcgatatccagcacactggcggccgttactagtggatccggctgctaacaaagcccgaaaggaagctgagttggctgctgccaccgctgagcaataactagcataaccccttggggcctctaaacgggtcttgaggggttttttgctgaaaggaggaactatatccggagcgactcccacggcacgttggcaagctcg

SEQ ID NO: 80 - DNA, 1400 bp, Artificial Sequence
  Exemplary msLacBP6.50C expression sequence.
cggtcacgcttgggactgccataggctggcccggtgatgccggccacgatgcgtccggcgtagaggatcgagatctcgatcccgcgaaattaatacgactcactatagggagaccacaacggtttccctctagaaataattttgtttaactttaagaaggagatataccatggcaacaacttggaaaattcaaagtgtatgggatgcagggacggtgggctatgacctcttcaaggagtggagcgacggtatggaagaaaagacgggcggtgaactcaaattcacggcgttcccagccaaagccgtcgccgcagattgtaatggtctttttgatgcagtacggaatggcgtcttgcaaggtatgaatcctttcaccctctactggtcaggtaagattccggcctccgtatttctctcgtcgtacccagccggtccagatcaaccacatcaatgggatacaatgttctacagccttggtatgttagaaaaaacacgtgaaatttacaaaaagttcggcctcttctacgtcggcccaattcagcacgacgcaaacattatccacagtaaacagccgattaattccctggacgaccttaagggtctcaaaatgcgcttacctggcgggatggtagcggaagtctttgcaaagtttggcgtcgcagcggtcagtctcccaggcagcgacatctttccagccttagaaaaaggcacaatcgacgctgctgattacgtgggtccggctgtaaactgggagctcggcttcagccaagtaacaaagtacatcttaatgggtccaccaggcatcatgtcagtctaccaaccggtcgaccttatggacctcactgtcaatctgcgggcctggaacgcattagatccaaagttacagcaaatcgttgaagatgaagtacgcatctactctcagaagcattacctcgcaattcagaaacggaatattgaagctatgaagaagttcgaggccgctggtacaaccgtaacccgtctgtcacaagaggacctccaggagtttcgtcgtgcagctatcccaatttggtattcatgggcaaacaaagatgaagacgcacgggagattttcgacatgcaattagagtacatgatgaacgacactgtaggttacatcactgaagatgacattaagggcatgaatggcggttcacatcatcatcatcatcattaatgaaagggcgatatccagcacactggcggccgttactagtggatccggctgctaacaaagcccgaaaggaagctgagttggctgctgccaccgctgagcaataactagcataaccccttggggcctctaaacgggtcttgaggggttttttgctgaaaggaggaactatatccggagcgactcccacggcacgttggcaagctcg

SEQ ID NO: 81 - DNA, 1400 bp, Artificial Sequence
  Exemplary msLacBP6.68C expression sequence.
cggtcacgcttgggactgccataggctggcccggtgatgccggccacgatgcgtccggcgtagaggatcgagatctcgatcccgcgaaattaatacgactcactatagggagaccacaacggtttccctctagaaataattttgtttaactttaagaaggagatataccatggcaacaacttggaaaattcaaagtgtatgggatgcagggacggtgggctatgacctcttcaaggagtggagcgacggtatggaagaaaagacgggcggtgaactcaaattcacggcgttcccagccaaagccgtcgccgcagataataatggtctttttgatgcagtacggaatggcgtcttgcaaggtatgaatccttgtaccctctactggtcaggtaagattccggcctccgtatttctctcgtcgtacccagccggtccagatcaaccacatcaatgggatacaatgttctacagccttggtatgttagaaaaaacacgtgaaatttacaaaaagttcggcctcttctacgtcggcccaattcagcacgacgcaaacattatccacagtaaacagccgattaattccctggacgaccttaagggtctcaaaatgcgcttacctggcgggatggtagcggaagtctttgcaaagtttggcgtcgcagcggtcagtctcccaggcagcgacatctttccagccttagaaaaaggcacaatcgacgctgctgattacgtgggtccggctgtaaactgggagctcggcttcagccaagtaacaaagtacatcttaatgggtccaccaggcatcatgtcagtctaccaaccggtcgaccttatggacctcactgtcaatctgcgggcctggaacgcattagatccaaagttacagcaaatcgttgaagatgaagtacgcatctactctcagaagcattacctcgcaattcagaaacggaatattgaagctatgaagaagttcgaggccgctggtacaaccgtaacccgtctgtcacaagaggacctccaggagtttcgtcgtgcagctatcccaatttggtattcatgggcaaacaaagatgaagacgcacgggagattttcgacatgcaattagagtacatgatgaacgacactgtaggttacatcactgaagatgacattaagggcatgaatggcggttcacatcatcatcatcatcattaatgaaagggcgatatccagcacactggcggccgttactagtggatccggctgctaacaaagcccgaaaggaagctgagttggctgctgccaccgctgagcaataactagcataaccccttggggcctctaaacgggtcttgaggggttttttgctgaaaggaggaactatatccggagcgactcccacggcacgttggcaagctcg

SEQ ID NO: 82 - DNA, 1400 bp, Artificial Sequence
  Exemplary msLacBP6.169C  expression sequence.
cggtcacgcttgggactgccataggctggcccggtgatgccggccacgatgcgtccggcgtagaggatcgagatctcgatcccgcgaaattaatacgactcactatagggagaccacaacggtttccctctagaaataattttgtttaactttaagaaggagatataccatggcaacaacttggaaaattcaaagtgtatgggatgcagggacggtgggctatgacctcttcaaggagtggagcgacggtatggaagaaaagacgggcggtgaactcaaattcacggcgttcccagccaaagccgtcgccgcagataataatggtctttttgatgcagtacggaatggcgtcttgcaaggtatgaatcctttcaccctctactggtcaggtaagattccggcctccgtatttctctcgtcgtacccagccggtccagatcaaccacatcaatgggatacaatgttctacagccttggtatgttagaaaaaacacgtgaaatttacaaaaagttcggcctcttctacgtcggcccaattcagcacgacgcaaacattatccacagtaaacagccgattaattccctggacgaccttaagggtctcaaaatgcgcttacctggcgggatggtagcggaagtctttgcaaagtttggcgtcgcagcggtcagtctctgtggcagcgacatctttccagccttagaaaaaggcacaatcgacgctgctgattacgtgggtccggctgtaaactgggagctcggcttcagccaagtaacaaagtacatcttaatgggtccaccaggcatcatgtcagtctaccaaccggtcgaccttatggacctcactgtcaatctgcgggcctggaacgcattagatccaaagttacagcaaatcgttgaagatgaagtacgcatctactctcagaagcattacctcgcaattcagaaacggaatattgaagctatgaagaagttcgaggccgctggtacaaccgtaacccgtctgtcacaagaggacctccaggagtttcgtcgtgcagctatcccaatttggtattcatgggcaaacaaagatgaagacgcacgggagattttcgacatgcaattagagtacatgatgaacgacactgtaggttacatcactgaagatgacattaagggcatgaatggcggttcacatcatcatcatcatcattaatgaaagggcgatatccagcacactggcggccgttactagtggatccggctgctaacaaagcccgaaaggaagctgagttggctgctgccaccgctgagcaataactagcataaccccttggggcctctaaacgggtcttgaggggttttttgctgaaaggaggaactatatccggagcgactcccacggcacgttggcaagctcg

SEQ ID NO: 83 - DNA, 1400 bp, Artificial Sequence
  Exemplary msLacBP6.170C expression sequence.
cggtcacgcttgggactgccataggctggcccggtgatgccggccacgatgcgtccggcgtagaggatcgagatctcgatcccgcgaaattaatacgactcactatagggagaccacaacggtttccctctagaaataattttgtttaactttaagaaggagatataccatggcaacaacttggaaaattcaaagtgtatgggatgcagggacggtgggctatgacctcttcaaggagtggagcgacggtatggaagaaaagacgggcggtgaactcaaattcacggcgttcccagccaaagccgtcgccgcagataataatggtctttttgatgcagtacggaatggcgtcttgcaaggtatgaatcctttcaccctctactggtcaggtaagattccggcctccgtatttctctcgtcgtacccagccggtccagatcaaccacatcaatgggatacaatgttctacagccttggtatgttagaaaaaacacgtgaaatttacaaaaagttcggcctcttctacgtcggcccaattcagcacgacgcaaacattatccacagtaaacagccgattaattccctggacgaccttaagggtctcaaaatgcgcttacctggcgggatggtagcggaagtctttgcaaagtttggcgtcgcagcggtcagtctcccatgtagcgacatctttccagccttagaaaaaggcacaatcgacgctgctgattacgtgggtccggctgtaaactgggagctcggcttcagccaagtaacaaagtacatcttaatgggtccaccaggcatcatgtcagtctaccaaccggtcgaccttatggacctcactgtcaatctgcgggcctggaacgcattagatccaaagttacagcaaatcgttgaagatgaagtacgcatctactctcagaagcattacctcgcaattcagaaacggaatattgaagctatgaagaagttcgaggccgctggtacaaccgtaacccgtctgtcacaagaggacctccaggagtttcgtcgtgcagctatcccaatttggtattcatgggcaaacaaagatgaagacgcacgggagattttcgacatgcaattagagtacatgatgaacgacactgtaggttacatcactgaagatgacattaagggcatgaatggcggttcacatcatcatcatcatcattaatgaaagggcgatatccagcacactggcggccgttactagtggatccggctgctaacaaagcccgaaaggaagctgagttggctgctgccaccgctgagcaataactagcataaccccttggggcctctaaacgggtcttgaggggttttttgctgaaaggaggaactatatccggagcgactcccacggcacgttggcaagctcg

SEQ ID NO: 84 - DNA, 1400 bp, Artificial Sequence
  Exemplary msLacBP6.171C expression sequence.
cggtcacgcttgggactgccataggctggcccggtgatgccggccacgatgcgtccggcgtagaggatcgagatctcgatcccgcgaaattaatacgactcactatagggagaccacaacggtttccctctagaaataattttgtttaactttaagaaggagatataccatggcaacaacttggaaaattcaaagtgtatgggatgcagggacggtgggctatgacctcttcaaggagtggagcgacggtatggaagaaaagacgggcggtgaactcaaattcacggcgttcccagccaaagccgtcgccgcagataataatggtctttttgatgcagtacggaatggcgtcttgcaaggtatgaatcctttcaccctctactggtcaggtaagattccggcctccgtatttctctcgtcgtacccagccggtccagatcaaccacatcaatgggatacaatgttctacagccttggtatgttagaaaaaacacgtgaaatttacaaaaagttcggcctcttctacgtcggcccaattcagcacgacgcaaacattatccacagtaaacagccgattaattccctggacgaccttaagggtctcaaaatgcgcttacctggcgggatggtagcggaagtctttgcaaagtttggcgtcgcagcggtcagtctcccaggctgtgacatctttccagccttagaaaaaggcacaatcgacgctgctgattacgtgggtccggctgtaaactgggagctcggcttcagccaagtaacaaagtacatcttaatgggtccaccaggcatcatgtcagtctaccaaccggtcgaccttatggacctcactgtcaatctgcgggcctggaacgcattagatccaaagttacagcaaatcgttgaagatgaagtacgcatctactctcagaagcattacctcgcaattcagaaacggaatattgaagctatgaagaagttcgaggccgctggtacaaccgtaacccgtctgtcacaagaggacctccaggagtttcgtcgtgcagctatcccaatttggtattcatgggcaaacaaagatgaagacgcacgggagattttcgacatgcaattagagtacatgatgaacgacactgtaggttacatcactgaagatgacattaagggcatgaatggcggttcacatcatcatcatcatcattaatgaaagggcgatatccagcacactggcggccgttactagtggatccggctgctaacaaagcccgaaaggaagctgagttggctgctgccaccgctgagcaataactagcataaccccttggggcctctaaacgggtcttgaggggttttttgctgaaaggaggaactatatccggagcgactcccacggcacgttggcaagctcg

SEQ ID NO: 85 - DNA, 1400 bp, Artificial Sequence
  Exemplary msLacBP6.187C expression sequence.
cggtcacgcttgggactgccataggctggcccggtgatgccggccacgatgcgtccggcgtagaggatcgagatctcgatcccgcgaaattaatacgactcactatagggagaccacaacggtttccctctagaaataattttgtttaactttaagaaggagatataccatggcaacaacttggaaaattcaaagtgtatgggatgcagggacggtgggctatgacctcttcaaggagtggagcgacggtatggaagaaaagacgggcggtgaactcaaattcacggcgttcccagccaaagccgtcgccgcagataataatggtctttttgatgcagtacggaatggcgtcttgcaaggtatgaatcctttcaccctctactggtcaggtaagattccggcctccgtatttctctcgtcgtacccagccggtccagatcaaccacatcaatgggatacaatgttctacagccttggtatgttagaaaaaacacgtgaaatttacaaaaagttcggcctcttctacgtcggcccaattcagcacgacgcaaacattatccacagtaaacagccgattaattccctggacgaccttaagggtctcaaaatgcgcttacctggcgggatggtagcggaagtctttgcaaagtttggcgtcgcagcggtcagtctcccaggcagcgacatctttccagccttagaaaaaggcacaatcgacgctgctgattgtgtgggtccggctgtaaactgggagctcggcttcagccaagtaacaaagtacatcttaatgggtccaccaggcatcatgtcagtctaccaaccggtcgaccttatggacctcactgtcaatctgcgggcctggaacgcattagatccaaagttacagcaaatcgttgaagatgaagtacgcatctactctcagaagcattacctcgcaattcagaaacggaatattgaagctatgaagaagttcgaggccgctggtacaaccgtaacccgtctgtcacaagaggacctccaggagtttcgtcgtgcagctatcccaatttggtattcatgggcaaacaaagatgaagacgcacgggagattttcgacatgcaattagagtacatgatgaacgacactgtaggttacatcactgaagatgacattaagggcatgaatggcggttcacatcatcatcatcatcattaatgaaagggcgatatccagcacactggcggccgttactagtggatccggctgctaacaaagcccgaaaggaagctgagttggctgctgccaccgctgagcaataactagcataaccccttggggcctctaaacgggtcttgaggggttttttgctgaaaggaggaactatatccggagcgactcccacggcacgttggcaagctcg

SEQ ID NO: 86 - DNA, 1400 bp, Artificial Sequence
  Exemplary msLacBP6.188C expression sequence.
cggtcacgcttgggactgccataggctggcccggtgatgccggccacgatgcgtccggcgtagaggatcgagatctcgatcccgcgaaattaatacgactcactatagggagaccacaacggtttccctctagaaataattttgtttaactttaagaaggagatataccatggcaacaacttggaaaattcaaagtgtatgggatgcagggacggtgggctatgacctcttcaaggagtggagcgacggtatggaagaaaagacgggcggtgaactcaaattcacggcgttcccagccaaagccgtcgccgcagataataatggtctttttgatgcagtacggaatggcgtcttgcaaggtatgaatcctttcaccctctactggtcaggtaagattccggcctccgtatttctctcgtcgtacccagccggtccagatcaaccacatcaatgggatacaatgttctacagccttggtatgttagaaaaaacacgtgaaatttacaaaaagttcggcctcttctacgtcggcccaattcagcacgacgcaaacattatccacagtaaacagccgattaattccctggacgaccttaagggtctcaaaatgcgcttacctggcgggatggtagcggaagtctttgcaaagtttggcgtcgcagcggtcagtctcccaggcagcgacatctttccagccttagaaaaaggcacaatcgacgctgctgattactgtggtccggctgtaaactgggagctcggcttcagccaagtaacaaagtacatcttaatgggtccaccaggcatcatgtcagtctaccaaccggtcgaccttatggacctcactgtcaatctgcgggcctggaacgcattagatccaaagttacagcaaatcgttgaagatgaagtacgcatctactctcagaagcattacctcgcaattcagaaacggaatattgaagctatgaagaagttcgaggccgctggtacaaccgtaacccgtctgtcacaagaggacctccaggagtttcgtcgtgcagctatcccaatttggtattcatgggcaaacaaagatgaagacgcacgggagattttcgacatgcaattagagtacatgatgaacgacactgtaggttacatcactgaagatgacattaagggcatgaatggcggttcacatcatcatcatcatcattaatgaaagggcgatatccagcacactggcggccgttactagtggatccggctgctaacaaagcccgaaaggaagctgagttggctgctgccaccgctgagcaataactagcataaccccttggggcctctaaacgggtcttgaggggttttttgctgaaaggaggaactatatccggagcgactcccacggcacgttggcaagctcg

SEQ ID NO: 87 - DNA, 1400 bp, Artificial Sequence
  Exemplary msLacBP6.192C expression sequence.
cggtcacgcttgggactgccataggctggcccggtgatgccggccacgatgcgtccggcgtagaggatcgagatctcgatcccgcgaaattaatacgactcactatagggagaccacaacggtttccctctagaaataattttgtttaactttaagaaggagatataccatggcaacaacttggaaaattcaaagtgtatgggatgcagggacggtgggctatgacctcttcaaggagtggagcgacggtatggaagaaaagacgggcggtgaactcaaattcacggcgttcccagccaaagccgtcgccgcagataataatggtctttttgatgcagtacggaatggcgtcttgcaaggtatgaatcctttcaccctctactggtcaggtaagattccggcctccgtatttctctcgtcgtacccagccggtccagatcaaccacatcaatgggatacaatgttctacagccttggtatgttagaaaaaacacgtgaaatttacaaaaagttcggcctcttctacgtcggcccaattcagcacgacgcaaacattatccacagtaaacagccgattaattccctggacgaccttaagggtctcaaaatgcgcttacctggcgggatggtagcggaagtctttgcaaagtttggcgtcgcagcggtcagtctcccaggcagcgacatctttccagccttagaaaaaggcacaatcgacgctgctgattacgtgggtccggcttgtaactgggagctcggcttcagccaagtaacaaagtacatcttaatgggtccaccaggcatcatgtcagtctaccaaccggtcgaccttatggacctcactgtcaatctgcgggcctggaacgcattagatccaaagttacagcaaatcgttgaagatgaagtacgcatctactctcagaagcattacctcgcaattcagaaacggaatattgaagctatgaagaagttcgaggccgctggtacaaccgtaacccgtctgtcacaagaggacctccaggagtttcgtcgtgcagctatcccaatttggtattcatgggcaaacaaagatgaagacgcacgggagattttcgacatgcaattagagtacatgatgaacgacactgtaggttacatcactgaagatgacattaagggcatgaatggcggttcacatcatcatcatcatcattaatgaaagggcgatatccagcacactggcggccgttactagtggatccggctgctaacaaagcccgaaaggaagctgagttggctgctgccaccgctgagcaataactagcataaccccttggggcctctaaacgggtcttgaggggttttttgctgaaaggaggaactatatccggagcgactcccacggcacgttggcaagctcg

SEQ ID NO: 88 - DNA, 1400 bp, Artificial Sequence
  Exemplary msLacBP6.196C expression sequence.
cggtcacgcttgggactgccataggctggcccggtgatgccggccacgatgcgtccggcgtagaggatcgagatctcgatcccgcgaaattaatacgactcactatagggagaccacaacggtttccctctagaaataattttgtttaactttaagaaggagatataccatggcaacaacttggaaaattcaaagtgtatgggatgcagggacggtgggctatgacctcttcaaggagtggagcgacggtatggaagaaaagacgggcggtgaactcaaattcacggcgttcccagccaaagccgtcgccgcagataataatggtctttttgatgcagtacggaatggcgtcttgcaaggtatgaatcctttcaccctctactggtcaggtaagattccggcctccgtatttctctcgtcgtacccagccggtccagatcaaccacatcaatgggatacaatgttctacagccttggtatgttagaaaaaacacgtgaaatttacaaaaagttcggcctcttctacgtcggcccaattcagcacgacgcaaacattatccacagtaaacagccgattaattccctggacgaccttaagggtctcaaaatgcgcttacctggcgggatggtagcggaagtctttgcaaagtttggcgtcgcagcggtcagtctcccaggcagcgacatctttccagccttagaaaaaggcacaatcgacgctgctgattacgtgggtccggctgtaaactgggagtgtggcttcagccaagtaacaaagtacatcttaatgggtccaccaggcatcatgtcagtctaccaaccggtcgaccttatggacctcactgtcaatctgcgggcctggaacgcattagatccaaagttacagcaaatcgttgaagatgaagtacgcatctactctcagaagcattacctcgcaattcagaaacggaatattgaagctatgaagaagttcgaggccgctggtacaaccgtaacccgtctgtcacaagaggacctccaggagtttcgtcgtgcagctatcccaatttggtattcatgggcaaacaaagatgaagacgcacgggagattttcgacatgcaattagagtacatgatgaacgacactgtaggttacatcactgaagatgacattaagggcatgaatggcggttcacatcatcatcatcatcattaatgaaagggcgatatccagcacactggcggccgttactagtggatccggctgctaacaaagcccgaaaggaagctgagttggctgctgccaccgctgagcaataactagcataaccccttggggcctctaaacgggtcttgaggggttttttgctgaaaggaggaactatatccggagcgactcccacggcacgttggcaagctcg

SEQ ID NO: 89 - DNA, 1406 bp, Artificial Sequence
  Exemplary tsLacBP7.189C expression sequence.
cggtcacgcttgggactgccataggctggcccggtgatgccggccacgatgcgtccggcgtagaggatcgagatctcgatcccgcgaaattaatacgactcactatagggagaccacaacggtttccctctagaaataattttgtttaactttaagaaggagatataccatgcaagcaccacgttttcgttggcgtattcaaagtgcatgggatgcaggaacagtgggttacaccctctttcagcgctttgcagaacgcgtcaaagagctgaccgatggacagatcgagatccagacctttccagcgggtgcagtcgtgggtaccttcgacatgttcgacgcagtcaaaaccggagtgctggatggcatgcatccctttaccctctattgggcaggtcgaatgccggttaccgcctttctcagcagctacccgttaggcctggatcgaccagatcagtgggaaacgtggtactacgcacttggcggtctggatctggcgagacgtgcattcgaggaacagggtctgttctacgttggtccagtgcagcatgactacaacctgatccacagcaaaaagccgatcaagtccttcgaggacttcaaaggcgtgaagctgagagtgcctggtggcatgatagcagacgtcttctcagcagctggagcagcaacagtcctcttgcctggtggtgaggtctatccggctctggaacgtggtgtgatcgatgcagcagactgcgtgggtcctgcagtgaactacaaccttggcttccatcaggtgaccaagtacatcatcatgggtcctccagaaacccctgcgatccatcagccagtggatctggcagacatcaccctgaacctcagccgttggcgtgcagtgcccaaaaacctgcaggaacgattcgaagcagcggttcacgaatggagctggatccactatgccggtatccagaaagccaacctggagacctggccgaagtacaaagcggcaggtgtgcagatcatcaggctgactaccgtggatgtgcgcaagtttcgtcgtgttgcgattccgatctggttcaaatgggcgaaacaggacaagtatgcccgtgaagcctttgcaagccagctggagtacatgaaagcactgggctatgtgacagatgcagatgttcgtggtttaagcttaggcggcagccatcatcatcatcatcattaataatgaaagggcgatatccagcacactggcggccgttactagtggatccggctgctaacaaagcccgaaaggaagctgagttggctgctgccaccgctgagcaataactagcataaccccttggggcctctaaacgggtcttgaggggttttttgctgaaaggaggaactatatccggagcgactcccacggcacgttggcaagctcg

SEQ ID NO: 90 - DNA, 1406 bp, Artificial Sequence
  Exemplary maLacBP8.189C expression sequence.
cggtcacgcttgggactgccataggctggcccggtgatgccggccacgatgcgtccggcgtagaggatcgagatctcgatcccgcgaaattaatacgactcactatagggagaccacaacggtttccctctagaaataattttgtttaactttaagaaggagatataccatgcaagcagcaactacttggaaaattcaaagtacctgggatgctggtacggttggctacaccctcttcgaagagtgggcgaagagcatcgaagccaaatccggtggtgaactgaagttccaggcgtttccggcaaaagccgttgctgctgacaacaacgcgctctttgacgctgttcgcaacggtgtgcttcagggcatgaacccgttcaccctgtactgggcgggcaaaatccctgcctctgtgttcctgtcgagctacccagcaggtccggatcaaccccatcagtgggataccatgttctactcgatgggtatgctggagaaaacccgcgaaatctacaagaaatttggcctgttctacgttggtccgatccagcatgatgcgaacatcatccacagcaaacagccagtcaactctctggacgacctgaaagggatgaagatccgtgtacctggtggcatggttgccgaagtcttccagcagtttggcgtttccaccgtcagtctgccgggtagcgacatcttcccggcattggagaaaggcacgattgacgctgcagactgcgtaggtccagcagtcaactacgaactgggctttagccaggttacggactacatcatcttcggaccacctggcgtcatgagcatctatcaaccggtggacctgatggatctgaccgtcagtctgcgtgcttggaactcgatctcaccagagctgcagcagctggttgaggatgaagtgcgcatctactcgcagaaacactatctggcgattcaggctcgcaacatcgaagcgatggagaaattcaaagccgatggtgacacggtaacccgtctgagccaggaagacctggaaacctggcgtaaggctgcaatcccgatctggttcaactgggcgaacaagaacgatgatgctcgtgcgatcctggatatccagctgaaatacatgatgaacgacactgtgggctacattactgaagaagatattaaaggatttggcggcagccatcatcatcatcatcattaatgataaaagggcgatatccagcacactggcggccgttactagtggatccggctgctaacaaagcccgaaaggaagctgagttggctgctgccaccgctgagcaataactagcataaccccttggggcctctaaacgggtcttgaggggttttttgctgaaaggaggaactatatccggagcgactcccacggcacgttggcaagctcg

SEQ ID NO: 91 - DNA, 1439 bp, Artificial Sequence
  Exemplary adLacBP9.C191 expression sequence.
cggtcacgcttgggactgccataggctggcccggtgatgccggccacgatgcgtccggcgtagaggatcgagatctcgatcccgcgaaattaatacgactcactatagggagaccacaacggtttccctctagaaataattttgtttaactttaagaaggagatataccatgcaagcaccaattactctgagatttcagagtacttggccgcagaaagacatcttccacgagtttgccctggattacgccaaaaaggtcaacgagatgagcggtggacgtctgaagatcgaggttctggcagcaggcagtgtggtgaaggcgttcgatctcctggatgcagtgagcaagggtacgctggatggaggtcatggcgtagtcgcctactggtacggcaagaacaccgcattagcgctgtggggctctggacctgcattcggcatggacccaaacatggtgcttgcatggcaccattacggcggaggtcgtcagctcctggaagagatctaccgaagcctcaacctggatgtcgtcagcctcatgtacggaccaatgccgactcagccgttaggctggttcaagcagaaacccattgcgaaacctgacgacatgaaagggctgaagttccgtacggtaggtctgagcatcgacatcttcaacggactgggtgctgcagtgaacgcgttaccaggtgccgaaatcgttccggctatggatcgaggtctgctcgatgcggcagagtgcaacaacgcttcttccgatcgtgtgctagggtttccggatgtctcgaagatcgcgatgctgcaatcgttccatcaggcgtcagagcagttcgagatcctgttcaacggcaagcgtttccaggcgttaccggctgatctgaagagcatcatctccattgctgcgcaagctgcaagcgccgacatgtcctggaaggccatcgatcgctactctagcgactacttcgagatgcgtgacaagcagggcgtgaagttctacagcaccagaccggaaatcctgaaacggcaactggagatctgggaccaggtgatggagaagcgtgcagccgaaaacccgacgttcaaaaaggtcctggagagccaacgcaggtttgcacagcgtgctgcgagatggcagaacgacaccaacgtggacttcaagatggcctacaaccacttctttggtggtaagaaaaaagctactggcggcagccatcatcatcatcatcattaataatgaaagggcgatatccagcacactggcggccgttactagtggatccggctgctaacaaagcccgaaaggaagctgagttggctgctgccaccgctgagcaataactagcataaccccttggggcctctaaacgggtcttgaggggttttttgctgaaaggaggaactatatccggagcgactcccacggcacgttggcaagctcg

SEQ ID NO: 92 - DNA, 1415 bp, Artificial Sequence
  Exemplary psLacBP11.195C expression sequence.
cggtcacgcttgggactgccataggctggcccggtgatgccggccacgatgcgtccggcgtagaggatcgagatctcgatcccgcgaaattaatacgactcactatagggagaccacaacggtttccctctagaaataattttgtttaactttaagaaggagatataccatgcaacaagcagcaggtgaaccagcaaaaacctatcactggaagatggtgaccgcttggccgaagaactatccgggtttaggcaccagtgcggaacgactggcagaacgtgtgaacgcgatgagtggtggacgtctgaccatcaaggtgtatgcagcaggagaactggttccagctctggaagtgttcgatgcagtctctcgtggtaccgcagaactgggtcatggagcaagctactactggaaaggcaaggttccgactgcgcagttcttcaccagtgtaccgtttggtctgtcaaccagcgagatgaacgcatggctgagcaaaggtggtggacaggcgttctgggacgaagcctacgctcctttcggcgtgaaaccgcttgtgatcggcaataccggcatgcagatgggtggatggtacaacaaagagatcaacagcctgactgacctcaaaggcctgaaaatccgcatgccaggtctgggtggtgaagtgctaagcagactgggtgcaaccaccgtgaaccttccaggtggtgaagtctttaccgcactgcagacaggagcgatcgatgcaaccgattgcgtgagtccctacaacgatctggcctttggtctgcacaaagcagcacgctactactactacccgggttggcaggaaccacaggctgtactggaactgctgatcaaccagaaggcgttcgatagcttaccggcagatctgcaggcgatcgtgaccgaagcaagcctggcagcaagccgcgatatgcatgacgattacgtctacaacaacgctctggctctggaacagctcaaacagcagggaaccgaactgaagcgctttccggacgaagtgctggcagcaatgcgcgaacagtctgacctgatcctcggtgaactggctgcacagagcgaactgaacggtcgtatctgggcaagcatgaaggcctttcaggctcaggtcgaaccgatgcacgagattagcgaaaaagaattgtataattggagaggcggcagccatcatcatcatcatcattaataatgaaagggcgatatccagcacactggcggccgttactagtggatccggctgctaacaaagcccgaaaggaagctgagttggctgctgccaccgctgagcaataactagcataaccccttggggcctctaaacgggtcttgaggggttttttgctgaaaggaggaactatatccggagcgactcccacggcacgttggcaagctcg

SEQ ID NO: 93 - DNA, 1433 bp, Artificial Sequence
  Exemplary rsLacBP12.191C expression sequence.
cggtcacgcttgggactgccataggctggcccggtgatgccggccacgatgcgtccggcgtagaggatcgagatctcgatcccgcgaaattaatacgactcactatagggagaccacaacggtttccctctagaaataattttgtttaactttaagaaggagatataccatgcaagcaccgttagttatgaaaatgcaaactagttggccagctagcgatatctggatggacttcgcacgtgagtacgtgaccagagtggaagagatgtcaggtggacgcatcaaggtggatctgctgccagcaggtgcggtagttggtgcgttccaggtgatggacgcagtacacgatggggtcatcgatgctagccactcggtgagcgcttactggtatggcaagagcaaagcggctagcttctttggcactggtccagtctttggcggtagtgcaaccacgatgctcggctggttctaccaaggtggaggtcaggacctgtaccgtgaactgacgcaagacatcctcggaatgaacatcgtaggcttctacggtttcccgatgccggcacagccattcggctggttcaagacggaagtgaacggcgttgcggacatccaaggcttcaagtaccgtaccgttggactggcagcagatctgctgcaggctatgggcatgtcagtggcacagctgccaggtggcgaaatcgttccggcaatggagcgtggtgtgatcgatgcgttcgagtgcaacaaccctagctcggatatgcgctttggtgcacaagatgtggcgaagaactactacctgtcctcctaccatcaggcatctgagagcttcgagtacaccttcaatcgcgacttctacgaggatctggatcctgacctgcaagccatcctgaagtacgctgtggaagcagcgagtaccagcaataccgcgttagcgctgaggcagtatagcgcagatcttgcgacgttagcggctgaaaacggtgttgcagtgcatcggactccgaaagacatcctgtctggtcagctggaagcatgggacaagctgatcgtggatctcgaagcggatgagttcttcaagaaagtgctggattcccaacgtgcatgggtcgaacaggtctcctactacgagctgatgaacgcagcggatcttggactggcatacgaacatcattttccaggaaaattaaaactgggcggcagccatcatcatcatcatcattaataatgaaagggcgatatccagcacactggcggccgttactagtggatccggctgctaacaaagcccgaaaggaagctgagttggctgctgccaccgctgagcaataactagcataaccccttggggcctctaaacgggtcttgaggggttttttgctgaaaggaggaactatatccggagcgactcccacggcacgttggcaagctcg

SEQ ID NO: 94 - DNA, 1415 bp, Artificial Sequence
  Exemplary fsLacBP13.188C expression sequence.
cggtcacgcttgggactgccataggctggcccggtgatgccggccacgatgcgtccggcgtagaggatcgagatctcgatcccgcgaaattaatacgactcactatagggagaccacaacggtttccctctagaaataattttgtttaactttaagaaggagatataccatggaaaaaaaaattcgttggaaattagcaatgacttggggtccgaccttgcatccgttgtccgacacagcagagcatatggcggaaatcgtgaaggagttgagcgatggcaacttcgtgatcaacatcgatgcgtcgaacgtgcacaaagcgccgtttggcatcttcgatatggtgaaactcggtcagtacgagatgggccatactgcgagctactactacaaaggcaaaaacatcgcgtttttaccgctgacgaccatgcctttcggtatgaccgcaccggaacagtatgcgtggttctactatggtggcggtctggagctgatgcaggaagcgtacaccaagcatggcatgctggcgtttcctggtggtaacaccggtaaccagatgggaggttggttcaccaaggagatcaacagcctggatgacctcaagggtctcaagatgaggatcccaggctttgcgggccagatcatgtccaaactgggtgtgaccgtgaccaacatccctccaggtgagctgtacaccgcactggaacgtggtaccgtggatgcggtggaatgcaccggtcctggtatggacatcaacatgggattccacaagatcgcgaaatactactataccggttggcatgaaccgggatccgaagtggagttcctgatcaacgaaaaggaatacaacaaactgccggaaaaatacaaaaagatcctgaaaatcgccatgaaaaccgcagcgtacgacatgtacatccagtcgtacgagatgaacgctgaagcttggcagcagatgaaagagaaatacccggatatcaaggtcaaggtttttccggaagaagtgctgaaagagatgaagaccgcgtacgacaaccttgtggcgagctacgagaaagaaagcccgatgttcaagaaaatcatggagagcaaacgtgcgtatctggacaaggttcgagactggacccacatatcggactacctctacctgaaaagtacttctgaaagtaatctgaatggcggcagccatcatcatcatcatcattaatgataaaagggcgatatccagcacactggcggccgttactagtggatccggctgctaacaaagcccgaaaggaagctgagttggctgctgccaccgctgagcaataactagcataaccccttggggcctctaaacgggtcttgaggggttttttgctgaaaggaggaactatatccggagcgactcccacggcacgttggcaagctcg

SEQ ID NO: 95 - DNA, 1400 bp, Artificial Sequence
  Exemplary msLacBP6_187C_F68L expression sequence.
cggtcacgcttgggactgccataggctggcccggtgatgccggccacgatgcgtccggcgtagaggatcgagatctcgatcccgcgaaattaatacgactcactatagggagaccacaacggtttccctctagaaataattttgtttaactttaagaaggagatataccatggcaacaacttggaaaattcaaagtgtatgggatgcagggacggtgggctatgacctcttcaaggagtggtgcgacggtatggaagaaaagacgggcggtgaactcaaattcacgtgcttcccagccaaagccgtcgccgcagataataatggtctttttgatgcagtacggaatggcgtcttgcaaggtatgaatcctctgaccctctactggtcaggtaagattccggcctccgtatttctctcgtcgtacccagccggtccagatcaaccacatcaatgggatacaatgttctacagccttggtatgttagaaaaaacacgtgaaatttacaaaaagttcggcctcttctacgtcggcccaattcagcacgacgcaaacattatccacagtaaacagccgattaattccctggacgaccttaagggtctcaaaatgcgcttacctggcgggatggtagcggaagtctttgcaaagtttggcgtcgcagcggtcagtctcccaggcagcgacatctttccagccttagaaaaaggcacaatcgacgctgctgattgtgtgggtccggctgtaaactgggagctcggcttcagccaagtaacaaagtacatcttaatgggtccaccaggcatcatgtcagtctaccaaccggtcgaccttatggacctcactgtcaatctgcgggcctggaacgcattagatccaaagttacagcaaatcgttgaagatgaagtacgcatctactctcagaagcattacctcgcaattcagaaacggaatattgaagctatgaagaagttcgaggccgctggtacaaccgtaacccgtctgtcacaagaggacctccaggagtttcgtcgtgcagctatcccaatttggtattcatgggcaaacaaagatgaagacgcacgggagattttcgacatgcaattagagtacatgatgaacgacactgtaggttacatcactgaagatgacattaagggcatgaatggcggttcacatcatcatcatcatcattaatgaaagggcgatatccagcacactggcggccgttactagtggatccggctgctaacaaagcccgaaaggaagctgagttggctgctgccaccgctgagcaataactagcataaccccttggggcctctaaacgggtcttgaggggttttttgctgaaaggaggaactatatccggagcgactcccacggcacgttggcaagctcg

SEQ ID NO: 96 - DNA, 1400 bp, Artificial Sequence
  Exemplary msLacBP6_187C_F68M expression sequence.
cggtcacgcttgggactgccataggctggcccggtgatgccggccacgatgcgtccggcgtagaggatcgagatctcgatcccgcgaaattaatacgactcactatagggagaccacaacggtttccctctagaaataattttgtttaactttaagaaggagatataccatggcaacaacttggaaaattcaaagtgtatgggatgcagggacggtgggctatgacctcttcaaggagtggtgcgacggtatggaagaaaagacgggcggtgaactcaaattcacgtgcttcccagccaaagccgtcgccgcagataataatggtctttttgatgcagtacggaatggcgtcttgcaaggtatgaatcctatgaccctctactggtcaggtaagattccggcctccgtatttctctcgtcgtacccagccggtccagatcaaccacatcaatgggatacaatgttctacagccttggtatgttagaaaaaacacgtgaaatttacaaaaagttcggcctcttctacgtcggcccaattcagcacgacgcaaacattatccacagtaaacagccgattaattccctggacgaccttaagggtctcaaaatgcgcttacctggcgggatggtagcggaagtctttgcaaagtttggcgtcgcagcggtcagtctcccaggcagcgacatctttccagccttagaaaaaggcacaatcgacgctgctgattgtgtgggtccggctgtaaactgggagctcggcttcagccaagtaacaaagtacatcttaatgggtccaccaggcatcatgtcagtctaccaaccggtcgaccttatggacctcactgtcaatctgcgggcctggaacgcattagatccaaagttacagcaaatcgttgaagatgaagtacgcatctactctcagaagcattacctcgcaattcagaaacggaatattgaagctatgaagaagttcgaggccgctggtacaaccgtaacccgtctgtcacaagaggacctccaggagtttcgtcgtgcagctatcccaatttggtattcatgggcaaacaaagatgaagacgcacgggagattttcgacatgcaattagagtacatgatgaacgacactgtaggttacatcactgaagatgacattaagggcatgaatggcggttcacatcatcatcatcatcattaatgaaagggcgatatccagcacactggcggccgttactagtggatccggctgctaacaaagcccgaaaggaagctgagttggctgctgccaccgctgagcaataactagcataaccccttggggcctctaaacgggtcttgaggggttttttgctgaaaggaggaactatatccggagcgactcccacggcacgttggcaagctcg

SEQ ID NO: 97 - DNA, 1400 bp, Artificial Sequence
  Exemplary msLacBP6_187C_L70F expression sequence
cggtcacgcttgggactgccataggctggcccggtgatgccggccacgatgcgtccggcgtagaggatcgagatctcgatcccgcgaaattaatacgactcactatagggagaccacaacggtttccctctagaaataattttgtttaactttaagaaggagatataccatggcaacaacttggaaaattcaaagtgtatgggatgcagggacggtgggctatgacctcttcaaggagtggtgcgacggtatggaagaaaagacgggcggtgaactcaaattcacgtgcttcccagccaaagccgtcgccgcagataataatggtctttttgatgcagtacggaatggcgtcttgcaaggtatgaatcctttcaccttttactggtcaggtaagattccggcctccgtatttctctcgtcgtacccagccggtccagatcaaccacatcaatgggatacaatgttctacagccttggtatgttagaaaaaacacgtgaaatttacaaaaagttcggcctcttctacgtcggcccaattcagcacgacgcaaacattatccacagtaaacagccgattaattccctggacgaccttaagggtctcaaaatgcgcttacctggcgggatggtagcggaagtctttgcaaagtttggcgtcgcagcggtcagtctcccaggcagcgacatctttccagccttagaaaaaggcacaatcgacgctgctgattgtgtgggtccggctgtaaactgggagctcggcttcagccaagtaacaaagtacatcttaatgggtccaccaggcatcatgtcagtctaccaaccggtcgaccttatggacctcactgtcaatctgcgggcctggaacgcattagatccaaagttacagcaaatcgttgaagatgaagtacgcatctactctcagaagcattacctcgcaattcagaaacggaatattgaagctatgaagaagttcgaggccgctggtacaaccgtaacccgtctgtcacaagaggacctccaggagtttcgtcgtgcagctatcccaatttggtattcatgggcaaacaaagatgaagacgcacgggagattttcgacatgcaattagagtacatgatgaacgacactgtaggttacatcactgaagatgacattaagggcatgaatggcggttcacatcatcatcatcatcattaatgaaagggcgatatccagcacactggcggccgttactagtggatccggctgctaacaaagcccgaaaggaagctgagttggctgctgccaccgctgagcaataactagcataaccccttggggcctctaaacgggtcttgaggggttttttgctgaaaggaggaactatatccggagcgactcccacggcacgttggcaagctcg

SEQ ID NO: 98 - DNA, 1400 bp, Artificial Sequence
  Exemplary msLacBP6_187C_L70I expression sequence.
cggtcacgcttgggactgccataggctggcccggtgatgccggccacgatgcgtccggcgtagaggatcgagatctcgatcccgcgaaattaatacgactcactatagggagaccacaacggtttccctctagaaataattttgtttaactttaagaaggagatataccatggcaacaacttggaaaattcaaagtgtatgggatgcagggacggtgggctatgacctcttcaaggagtggtgcgacggtatggaagaaaagacgggcggtgaactcaaattcacgtgcttcccagccaaagccgtcgccgcagataataatggtctttttgatgcagtacggaatggcgtcttgcaaggtatgaatcctttcaccatttactggtcaggtaagattccggcctccgtatttctctcgtcgtacccagccggtccagatcaaccacatcaatgggatacaatgttctacagccttggtatgttagaaaaaacacgtgaaatttacaaaaagttcggcctcttctacgtcggcccaattcagcacgacgcaaacattatccacagtaaacagccgattaattccctggacgaccttaagggtctcaaaatgcgcttacctggcgggatggtagcggaagtctttgcaaagtttggcgtcgcagcggtcagtctcccaggcagcgacatctttccagccttagaaaaaggcacaatcgacgctgctgattgtgtgggtccggctgtaaactgggagctcggcttcagccaagtaacaaagtacatcttaatgggtccaccaggcatcatgtcagtctaccaaccggtcgaccttatggacctcactgtcaatctgcgggcctggaacgcattagatccaaagttacagcaaatcgttgaagatgaagtacgcatctactctcagaagcattacctcgcaattcagaaacggaatattgaagctatgaagaagttcgaggccgctggtacaaccgtaacccgtctgtcacaagaggacctccaggagtttcgtcgtgcagctatcccaatttggtattcatgggcaaacaaagatgaagacgcacgggagattttcgacatgcaattagagtacatgatgaacgacactgtaggttacatcactgaagatgacattaagggcatgaatggcggttcacatcatcatcatcatcattaatgaaagggcgatatccagcacactggcggccgttactagtggatccggctgctaacaaagcccgaaaggaagctgagttggctgctgccaccgctgagcaataactagcataaccccttggggcctctaaacgggtcttgaggggttttttgctgaaaggaggaactatatccggagcgactcccacggcacgttggcaagctcg

SEQ ID NO: 99 - DNA, 1400 bp, Artificial Sequence
  Exemplary msLacBP6_187C_L70M expression sequence.
cggtcacgcttgggactgccataggctggcccggtgatgccggccacgatgcgtccggcgtagaggatcgagatctcgatcccgcgaaattaatacgactcactatagggagaccacaacggtttccctctagaaataattttgtttaactttaagaaggagatataccatggcaacaacttggaaaattcaaagtgtatgggatgcagggacggtgggctatgacctcttcaaggagtggtgcgacggtatggaagaaaagacgggcggtgaactcaaattcacgtgcttcccagccaaagccgtcgccgcagataataatggtctttttgatgcagtacggaatggcgtcttgcaaggtatgaatcctttcaccatgtactggtcaggtaagattccggcctccgtatttctctcgtcgtacccagccggtccagatcaaccacatcaatgggatacaatgttctacagccttggtatgttagaaaaaacacgtgaaatttacaaaaagttcggcctcttctacgtcggcccaattcagcacgacgcaaacattatccacagtaaacagccgattaattccctggacgaccttaagggtctcaaaatgcgcttacctggcgggatggtagcggaagtctttgcaaagtttggcgtcgcagcggtcagtctcccaggcagcgacatctttccagccttagaaaaaggcacaatcgacgctgctgattgtgtgggtccggctgtaaactgggagctcggcttcagccaagtaacaaagtacatcttaatgggtccaccaggcatcatgtcagtctaccaaccggtcgaccttatggacctcactgtcaatctgcgggcctggaacgcattagatccaaagttacagcaaatcgttgaagatgaagtacgcatctactctcagaagcattacctcgcaattcagaaacggaatattgaagctatgaagaagttcgaggccgctggtacaaccgtaacccgtctgtcacaagaggacctccaggagtttcgtcgtgcagctatcccaatttggtattcatgggcaaacaaagatgaagacgcacgggagattttcgacatgcaattagagtacatgatgaacgacactgtaggttacatcactgaagatgacattaagggcatgaatggcggttcacatcatcatcatcatcattaatgaaagggcgatatccagcacactggcggccgttactagtggatccggctgctaacaaagcccgaaaggaagctgagttggctgctgccaccgctgagcaataactagcataaccccttggggcctctaaacgggtcttgaggggttttttgctgaaaggaggaactatatccggagcgactcccacggcacgttggcaagctcg

SEQ ID NO: 100 - DNA, 1400 bp, Artificial Sequence
  Exemplary msLacBP6_187C_P150A expression sequence.
cggtcacgcttgggactgccataggctggcccggtgatgccggccacgatgcgtccggcgtagaggatcgagatctcgatcccgcgaaattaatacgactcactatagggagaccacaacggtttccctctagaaataattttgtttaactttaagaaggagatataccatggcaacaacttggaaaattcaaagtgtatgggatgcagggacggtgggctatgacctcttcaaggagtggtgcgacggtatggaagaaaagacgggcggtgaactcaaattcacgtgcttcccagccaaagccgtcgccgcagataataatggtctttttgatgcagtacggaatggcgtcttgcaaggtatgaatcctttcaccctctactggtcaggtaagattccggcctccgtatttctctcgtcgtacccagccggtccagatcaaccacatcaatgggatacaatgttctacagccttggtatgttagaaaaaacacgtgaaatttacaaaaagttcggcctcttctacgtcggcccaattcagcacgacgcaaacattatccacagtaaacagccgattaattccctggacgaccttaagggtctcaaaatgcgcttagcgggcgggatggtagcggaagtctttgcaaagtttggcgtcgcagcggtcagtctcccaggcagcgacatctttccagccttagaaaaaggcacaatcgacgctgctgattgtgtgggtccggctgtaaactgggagctcggcttcagccaagtaacaaagtacatcttaatgggtccaccaggcatcatgtcagtctaccaaccggtcgaccttatggacctcactgtcaatctgcgggcctggaacgcattagatccaaagttacagcaaatcgttgaagatgaagtacgcatctactctcagaagcattacctcgcaattcagaaacggaatattgaagctatgaagaagttcgaggccgctggtacaaccgtaacccgtctgtcacaagaggacctccaggagtttcgtcgtgcagctatcccaatttggtattcatgggcaaacaaagatgaagacgcacgggagattttcgacatgcaattagagtacatgatgaacgacactgtaggttacatcactgaagatgacattaagggcatgaatggcggttcacatcatcatcatcatcattaatgaaagggcgatatccagcacactggcggccgttactagtggatccggctgctaacaaagcccgaaaggaagctgagttggctgctgccaccgctgagcaataactagcataaccccttggggcctctaaacgggtcttgaggggttttttgctgaaaggaggaactatatccggagcgactcccacggcacgttggcaagctcg

SEQ ID NO: 101 - DNA, 1400 bp, Artificial Sequence
  Exemplary msLacBP6_187C_P150S expression sequence.
cggtcacgcttgggactgccataggctggcccggtgatgccggccacgatgcgtccggcgtagaggatcgagatctcgatcccgcgaaattaatacgactcactatagggagaccacaacggtttccctctagaaataattttgtttaactttaagaaggagatataccatggcaacaacttggaaaattcaaagtgtatgggatgcagggacggtgggctatgacctcttcaaggagtggtgcgacggtatggaagaaaagacgggcggtgaactcaaattcacgtgcttcccagccaaagccgtcgccgcagataataatggtctttttgatgcagtacggaatggcgtcttgcaaggtatgaatcctttcaccctctactggtcaggtaagattccggcctccgtatttctctcgtcgtacccagccggtccagatcaaccacatcaatgggatacaatgttctacagccttggtatgttagaaaaaacacgtgaaatttacaaaaagttcggcctcttctacgtcggcccaattcagcacgacgcaaacattatccacagtaaacagccgattaattccctggacgaccttaagggtctcaaaatgcgcttaagcggcgggatggtagcggaagtctttgcaaagtttggcgtcgcagcggtcagtctcccaggcagcgacatctttccagccttagaaaaaggcacaatcgacgctgctgattgtgtgggtccggctgtaaactgggagctcggcttcagccaagtaacaaagtacatcttaatgggtccaccaggcatcatgtcagtctaccaaccggtcgaccttatggacctcactgtcaatctgcgggcctggaacgcattagatccaaagttacagcaaatcgttgaagatgaagtacgcatctactctcagaagcattacctcgcaattcagaaacggaatattgaagctatgaagaagttcgaggccgctggtacaaccgtaacccgtctgtcacaagaggacctccaggagtttcgtcgtgcagctatcccaatttggtattcatgggcaaacaaagatgaagacgcacgggagattttcgacatgcaattagagtacatgatgaacgacactgtaggttacatcactgaagatgacattaagggcatgaatggcggttcacatcatcatcatcatcattaatgaaagggcgatatccagcacactggcggccgttactagtggatccggctgctaacaaagcccgaaaggaagctgagttggctgctgccaccgctgagcaataactagcataaccccttggggcctctaaacgggtcttgaggggttttttgctgaaaggaggaactatatccggagcgactcccacggcacgttggcaagctcg

SEQ ID NO: 102 - DNA, 1400 bp, Artificial Sequence
  Exemplary msLacBP6_187C_D220E expression sequence.
cggtcacgcttgggactgccataggctggcccggtgatgccggccacgatgcgtccggcgtagaggatcgagatctcgatcccgcgaaattaatacgactcactatagggagaccacaacggtttccctctagaaataattttgtttaactttaagaaggagatataccatggcaacaacttggaaaattcaaagtgtatgggatgcagggacggtgggctatgacctcttcaaggagtggtgcgacggtatggaagaaaagacgggcggtgaactcaaattcacgtgcttcccagccaaagccgtcgccgcagataataatggtctttttgatgcagtacggaatggcgtcttgcaaggtatgaatcctttcaccctctactggtcaggtaagattccggcctccgtatttctctcgtcgtacccagccggtccagatcaaccacatcaatgggatacaatgttctacagccttggtatgttagaaaaaacacgtgaaatttacaaaaagttcggcctcttctacgtcggcccaattcagcacgacgcaaacattatccacagtaaacagccgattaattccctggacgaccttaagggtctcaaaatgcgcttacctggcgggatggtagcggaagtctttgcaaagtttggcgtcgcagcggtcagtctcccaggcagcgacatctttccagccttagaaaaaggcacaatcgacgctgctgattgtgtgggtccggctgtaaactgggagctcggcttcagccaagtaacaaagtacatcttaatgggtccaccaggcatcatgtcagtctaccaaccggtcgaacttatggacctcactgtcaatctgcgggcctggaacgcattagatccaaagttacagcaaatcgttgaagatgaagtacgcatctactctcagaagcattacctcgcaattcagaaacggaatattgaagctatgaagaagttcgaggccgctggtacaaccgtaacccgtctgtcacaagaggacctccaggagtttcgtcgtgcagctatcccaatttggtattcatgggcaaacaaagatgaagacgcacgggagattttcgacatgcaattagagtacatgatgaacgacactgtaggttacatcactgaagatgacattaagggcatgaatggcggttcacatcatcatcatcatcattaatgaaagggcgatatccagcacactggcggccgttactagtggatccggctgctaacaaagcccgaaaggaagctgagttggctgctgccaccgctgagcaataactagcataaccccttggggcctctaaacgggtcttgaggggttttttgctgaaaggaggaactatatccggagcgactcccacggcacgttggcaagctcg

SEQ ID NO: 103 - DNA, 1400 bp, Artificial Sequence
  Exemplary msLacBP6_187C_D220L expression sequence.
cggtcacgcttgggactgccataggctggcccggtgatgccggccacgatgcgtccggcgtagaggatcgagatctcgatcccgcgaaattaatacgactcactatagggagaccacaacggtttccctctagaaataattttgtttaactttaagaaggagatataccatggcaacaacttggaaaattcaaagtgtatgggatgcagggacggtgggctatgacctcttcaaggagtggtgcgacggtatggaagaaaagacgggcggtgaactcaaattcacgtgcttcccagccaaagccgtcgccgcagataataatggtctttttgatgcagtacggaatggcgtcttgcaaggtatgaatcctttcaccctctactggtcaggtaagattccggcctccgtatttctctcgtcgtacccagccggtccagatcaaccacatcaatgggatacaatgttctacagccttggtatgttagaaaaaacacgtgaaatttacaaaaagttcggcctcttctacgtcggcccaattcagcacgacgcaaacattatccacagtaaacagccgattaattccctggacgaccttaagggtctcaaaatgcgcttacctggcgggatggtagcggaagtctttgcaaagtttggcgtcgcagcggtcagtctcccaggcagcgacatctttccagccttagaaaaaggcacaatcgacgctgctgattgtgtgggtccggctgtaaactgggagctcggcttcagccaagtaacaaagtacatcttaatgggtccaccaggcatcatgtcagtctaccaaccggtcctgcttatggacctcactgtcaatctgcgggcctggaacgcattagatccaaagttacagcaaatcgttgaagatgaagtacgcatctactctcagaagcattacctcgcaattcagaaacggaatattgaagctatgaagaagttcgaggccgctggtacaaccgtaacccgtctgtcacaagaggacctccaggagtttcgtcgtgcagctatcccaatttggtattcatgggcaaacaaagatgaagacgcacgggagattttcgacatgcaattagagtacatgatgaacgacactgtaggttacatcactgaagatgacattaagggcatgaatggcggttcacatcatcatcatcatcattaatgaaagggcgatatccagcacactggcggccgttactagtggatccggctgctaacaaagcccgaaaggaagctgagttggctgctgccaccgctgagcaataactagcataaccccttggggcctctaaacgggtcttgaggggttttttgctgaaaggaggaactatatccggagcgactcccacggcacgttggcaagctcg

SEQ ID NO: 104 - DNA, 1400 bp, Artificial Sequence
  Exemplary msLacBP6_187C_D220N expression sequence.
cggtcacgcttgggactgccataggctggcccggtgatgccggccacgatgcgtccggcgtagaggatcgagatctcgatcccgcgaaattaatacgactcactatagggagaccacaacggtttccctctagaaataattttgtttaactttaagaaggagatataccatggcaacaacttggaaaattcaaagtgtatgggatgcagggacggtgggctatgacctcttcaaggagtggtgcgacggtatggaagaaaagacgggcggtgaactcaaattcacgtgcttcccagccaaagccgtcgccgcagataataatggtctttttgatgcagtacggaatggcgtcttgcaaggtatgaatcctttcaccctctactggtcaggtaagattccggcctccgtatttctctcgtcgtacccagccggtccagatcaaccacatcaatgggatacaatgttctacagccttggtatgttagaaaaaacacgtgaaatttacaaaaagttcggcctcttctacgtcggcccaattcagcacgacgcaaacattatccacagtaaacagccgattaattccctggacgaccttaagggtctcaaaatgcgcttacctggcgggatggtagcggaagtctttgcaaagtttggcgtcgcagcggtcagtctcccaggcagcgacatctttccagccttagaaaaaggcacaatcgacgctgctgattgtgtgggtccggctgtaaactgggagctcggcttcagccaagtaacaaagtacatcttaatgggtccaccaggcatcatgtcagtctaccaaccggtcaaccttatggacctcactgtcaatctgcgggcctggaacgcattagatccaaagttacagcaaatcgttgaagatgaagtacgcatctactctcagaagcattacctcgcaattcagaaacggaatattgaagctatgaagaagttcgaggccgctggtacaaccgtaacccgtctgtcacaagaggacctccaggagtttcgtcgtgcagctatcccaatttggtattcatgggcaaacaaagatgaagacgcacgggagattttcgacatgcaattagagtacatgatgaacgacactgtaggttacatcactgaagatgacattaagggcatgaatggcggttcacatcatcatcatcatcattaatgaaagggcgatatccagcacactggcggccgttactagtggatccggctgctaacaaagcccgaaaggaagctgagttggctgctgccaccgctgagcaataactagcataaccccttggggcctctaaacgggtcttgaggggttttttgctgaaaggaggaactatatccggagcgactcccacggcacgttggcaagctcg

SEQ ID NO: 105 - DNA, 1400 bp, Artificial Sequence
  Exemplary msLacBP6_187C_D220Q expression sequence.
cggtcacgcttgggactgccataggctggcccggtgatgccggccacgatgcgtccggcgtagaggatcgagatctcgatcccgcgaaattaatacgactcactatagggagaccacaacggtttccctctagaaataattttgtttaactttaagaaggagatataccatggcaacaacttggaaaattcaaagtgtatgggatgcagggacggtgggctatgacctcttcaaggagtggtgcgacggtatggaagaaaagacgggcggtgaactcaaattcacgtgcttcccagccaaagccgtcgccgcagataataatggtctttttgatgcagtacggaatggcgtcttgcaaggtatgaatcctttcaccctctactggtcaggtaagattccggcctccgtatttctctcgtcgtacccagccggtccagatcaaccacatcaatgggatacaatgttctacagccttggtatgttagaaaaaacacgtgaaatttacaaaaagttcggcctcttctacgtcggcccaattcagcacgacgcaaacattatccacagtaaacagccgattaattccctggacgaccttaagggtctcaaaatgcgcttacctggcgggatggtagcggaagtctttgcaaagtttggcgtcgcagcggtcagtctcccaggcagcgacatctttccagccttagaaaaaggcacaatcgacgctgctgattgtgtgggtccggctgtaaactgggagctcggcttcagccaagtaacaaagtacatcttaatgggtccaccaggcatcatgtcagtctaccaaccggtccagcttatggacctcactgtcaatctgcgggcctggaacgcattagatccaaagttacagcaaatcgttgaagatgaagtacgcatctactctcagaagcattacctcgcaattcagaaacggaatattgaagctatgaagaagttcgaggccgctggtacaaccgtaacccgtctgtcacaagaggacctccaggagtttcgtcgtgcagctatcccaatttggtattcatgggcaaacaaagatgaagacgcacgggagattttcgacatgcaattagagtacatgatgaacgacactgtaggttacatcactgaagatgacattaagggcatgaatggcggttcacatcatcatcatcatcattaatgaaagggcgatatccagcacactggcggccgttactagtggatccggctgctaacaaagcccgaaaggaagctgagttggctgctgccaccgctgagcaataactagcataaccccttggggcctctaaacgggtcttgaggggttttttgctgaaaggaggaactatatccggagcgactcccacggcacgttggcaagctcg

SEQ ID NO: 106 - DNA, 1400 bp, Artificial Sequence
  Exemplary msLacBP6_187C_D220S expression sequence.
cggtcacgcttgggactgccataggctggcccggtgatgccggccacgatgcgtccggcgtagaggatcgagatctcgatcccgcgaaattaatacgactcactatagggagaccacaacggtttccctctagaaataattttgtttaactttaagaaggagatataccatggcaacaacttggaaaattcaaagtgtatgggatgcagggacggtgggctatgacctcttcaaggagtggtgcgacggtatggaagaaaagacgggcggtgaactcaaattcacgtgcttcccagccaaagccgtcgccgcagataataatggtctttttgatgcagtacggaatggcgtcttgcaaggtatgaatcctttcaccctctactggtcaggtaagattccggcctccgtatttctctcgtcgtacccagccggtccagatcaaccacatcaatgggatacaatgttctacagccttggtatgttagaaaaaacacgtgaaatttacaaaaagttcggcctcttctacgtcggcccaattcagcacgacgcaaacattatccacagtaaacagccgattaattccctggacgaccttaagggtctcaaaatgcgcttacctggcgggatggtagcggaagtctttgcaaagtttggcgtcgcagcggtcagtctcccaggcagcgacatctttccagccttagaaaaaggcacaatcgacgctgctgattgtgtgggtccggctgtaaactgggagctcggcttcagccaagtaacaaagtacatcttaatgggtccaccaggcatcatgtcagtctaccaaccggtcagccttatggacctcactgtcaatctgcgggcctggaacgcattagatccaaagttacagcaaatcgttgaagatgaagtacgcatctactctcagaagcattacctcgcaattcagaaacggaatattgaagctatgaagaagttcgaggccgctggtacaaccgtaacccgtctgtcacaagaggacctccaggagtttcgtcgtgcagctatcccaatttggtattcatgggcaaacaaagatgaagacgcacgggagattttcgacatgcaattagagtacatgatgaacgacactgtaggttacatcactgaagatgacattaagggcatgaatggcggttcacatcatcatcatcatcattaatgaaagggcgatatccagcacactggcggccgttactagtggatccggctgctaacaaagcccgaaaggaagctgagttggctgctgccaccgctgagcaataactagcataaccccttggggcctctaaacgggtcttgaggggttttttgctgaaaggaggaactatatccggagcgactcccacggcacgttggcaagctcg

SEQ ID NO: 107 - DNA, 1463 bp, Artificial Sequence
  Exemplary msLacBP6_187C_bZifC expression sequence.
cggtcacgcttgggactgccataggctggcccggtgatgccggccacgatgcgtccggcgtagaggatcgagatctcgatcccgcgaaattaatacgactcactatagggagaccacaacggtttccctctagaaataattttgtttaactttaagaaggagatataccatggcaacaacttggaaaattcaaagtgtatgggatgcagggacggtgggctatgacctcttcaaggagtggtgcgacggtatggaagaaaagacgggcggtgaactcaaattcacgtgcttcccagccaaagccgtcgccgcagataataatggtctttttgatgcagtacggaatggcgtcttgcaaggtatgaatcctttcaccctctactggtcaggtaagattccggcctccgtatttctctcgtcgtacccagccggtccagatcaaccacatcaatgggatacaatgttctacagccttggtatgttagaaaaaacacgtgaaatttacaaaaagttcggcctcttctacgtcggcccaattcagcacgacgcaaacattatccacagtaaacagccgattaattccctggacgaccttaagggtctcaaaatgcgcttacctggcgggatggtagcggaagtctttgcaaagtttggcgtcgcagcggtcagtctcccaggcagcgacatctttccagccttagaaaaaggcacaatcgacgctgctgattgtgtgggtccggctgtaaactgggagctcggcttcagccaagtaacaaagtacatcttaatgggtccaccaggcatcatgtcagtctaccaaccggtcgaccttatggacctcactgtcaatctgcgggcctggaacgcattagatccaaagttacagcaaatcgttgaagatgaagtacgcatctactctcagaagcattacctcgcaattcagaaacggaatattgaagctatgaagaagttcgaggccgctggtacaaccgtaacccgtctgtcacaagaggacctccaggagtttcgtcgtgcagctatcccaatttggtattcatgggcaaacaaagatgaagacgcacgggagattttcgacatgcaattagagtacatgatgaacgacactgtaggttacatcactgaagatgacattaagggcatgaatggcggcagcaccggcgaaaaaccgtataaatgtccggaatgtggcaaaagctttagccgcagcggcggttcacatcatcatcatcatcattaatgaaagggcgatatccagcacactggcggccgttactagtggatccggctgctaacaaagcccgaaaggaagctgagttggctgctgccaccgctgagcaataactagcataaccccttggggcctctaaacgggtcttgaggggttttttgctgaaaggaggaactatatccggagcgactcccacggcacgttggcaagctcg

SEQ ID NO: 108 - DNA, 1463 bp, Artificial Sequence
  Exemplary msLacBP6_188C_bZifC expression sequence.
cggtcacgcttgggactgccataggctggcccggtgatgccggccacgatgcgtccggcgtagaggatcgagatctcgatcccgcgaaattaatacgactcactatagggagaccacaacggtttccctctagaaataattttgtttaactttaagaaggagatataccatggcaacaacttggaaaattcaaagtgtatgggatgcagggacggtgggctatgacctcttcaaggagtggtgcgacggtatggaagaaaagacgggcggtgaactcaaattcacgtgcttcccagccaaagccgtcgccgcagataataatggtctttttgatgcagtacggaatggcgtcttgcaaggtatgaatcctttcaccctctactggtcaggtaagattccggcctccgtatttctctcgtcgtacccagccggtccagatcaaccacatcaatgggatacaatgttctacagccttggtatgttagaaaaaacacgtgaaatttacaaaaagttcggcctcttctacgtcggcccaattcagcacgacgcaaacattatccacagtaaacagccgattaattccctggacgaccttaagggtctcaaaatgcgcttacctggcgggatggtagcggaagtctttgcaaagtttggcgtcgcagcggtcagtctcccaggcagcgacatctttccagccttagaaaaaggcacaatcgacgctgctgattactgtggtccggctgtaaactgggagctcggcttcagccaagtaacaaagtacatcttaatgggtccaccaggcatcatgtcagtctaccaaccggtcgaccttatggacctcactgtcaatctgcgggcctggaacgcattagatccaaagttacagcaaatcgttgaagatgaagtacgcatctactctcagaagcattacctcgcaattcagaaacggaatattgaagctatgaagaagttcgaggccgctggtacaaccgtaacccgtctgtcacaagaggacctccaggagtttcgtcgtgcagctatcccaatttggtattcatgggcaaacaaagatgaagacgcacgggagattttcgacatgcaattagagtacatgatgaacgacactgtaggttacatcactgaagatgacattaagggcatgaatggcggcagcaccggcgaaaaaccgtataaatgtccggaatgtggcaaaagctttagccgcagcggcggttcacatcatcatcatcatcattaatgaaagggcgatatccagcacactggcggccgttactagtggatccggctgctaacaaagcccgaaaggaagctgagttggctgctgccaccgctgagcaataactagcataaccccttggggcctctaaacgggtcttgaggggttttttgctgaaaggaggaactatatccggagcgactcccacggcacgttggcaagctcg

SEQ ID NO: 109 - protein, 18 aa, Artificial Sequence
  bZif
TGEKPYKCPECGKSFSRS

SEQ ID NO: 110 - protein, 32 aa, Artificial Sequence
  ZF-QNK
TGEKPYKCPECGKSFSRSDHLSRHQRTHQNKK

SEQ ID NO: 111 - protein, 6 aa, Artificial Sequence
  Hexahistidine Tag
HHHHHH

SEQ ID NO: 112 - protein, 6 aa, Artificial Sequence
  Hexalysine Tag
KKKKKK

SEQ ID NO: 113 - protein, 9 aa, Artificial Sequence
  GGSHHHHHH
GGSHHHHHH

SEQ ID NO: 114 - protein, 309 aa, Artificial Sequence
  E. coli GGBP (with signal peptide removed)
ADTRIGVTIYKYDDNFMSVVRKAIEQDAKAAPDVQLLMNDSQNDQSKQNDQIDVLLAKGVKALAINLVDPAAAGTVIEKARGQNVPVVFFNKEPSRKALDSYDKAYYVGTDSKESGIIQGDLIAKHWAANQGWDLNKDGQIQFVLLKGEPGHPDAEARTTYVIKELNDKGIKTEQLQLDTAMWDTAQAKDKMDAWLSGPNANKIEVVIANNDAMAMGAVEALKAHNKSSIPVFGVDALPEALALVKSGALAGTVLNDANNQAKATFDLAKNQADGKGAADGTNWKIDNKVVRVPYVGVDKDNLAEFSKK

SEQ ID NO: 115 - protein, 340 aa, Artificial Sequence
  ttLacPB1  (with signal peptide replaced with M)
MFSPLAVAQARRYRWRIQTAWDAGTVGYSLFQKFTERVKELTDGQLEVQPFPAGAVVGTFDMFDAVKTGVLDGMNPFTLYWAGRMPVTAFLSSYALGLDRPDQWETWFYSLGGLDIARRAFAEQGLFYVGPVQHDLNIIHSKKPIRRFEDFKGVKLRVPGGMIAEVFAAAGASTVLLPGGEVYPALERGVIDAADFVGPAVNYNLGFHQVAKYIIMGPPETPAIHQPVDLMDFTINLNRWRSLPKPLQERFIAAVHEYSWIHYAGIQKANLEAWPKYRQAGVEVIRLSNEDVRKFRRLAIPIWFKWAKMDKYSREAFASQLEYMKGIGYVTDEELKGLSL

SEQ ID NO: 116 - protein, 340 aa, Artificial Sequence
  tsLacBP2  (with signal peptide replaced with M)
MFSPLAVAQAPRFRWRIQSAWDAGTVGYSLFQKFAERVKELTDGQIEIQTFPAGAVVGTFDMFDAVKTGVLDGMHPFTLYWAGRMPVTAFLSSYPLGLDRPDQWETWYYGLGGLELARKAYEEQGLFFVGPVQHDYNLIHSKKPIKSFEDFKGVKLRVPGGMIAEIFAAAGAATVLLPGGEVYPALERGVIDAADFVGPAVNYNLGFHQVTKYIIMGPPETPAIHQPVDLADITININRWRALPRNLQERFEAAVHEWSWIHYAGIQKANLETWPKYKAAGVQVIRLSTVDVRKFRRVAIPIWFKWAKQDKYTREAFASQLEYMKALGYVTDADIRGLSL

SEQ ID NO: 117 - protein, 360 aa, Artificial Sequence
  toLacBP3  (with signal peptide replaced with M)
MKSTRRQFLKKAAIGVAASSAFSPLAIAQAPRFRWRIQSAWDAGTVGYTLFQRFAERVKELTDGQIEIQPFPAGAVVGTFDMFDAVKTGVLDGMHPFTLYWAGRMPVTAFLSSYPLGLDRPDQWETWYYGLGGLELARKAYEEQGLAYIGPVQHDYNLIHSKKPIKSFEEFKGVKLRVPGGMIAEIFAAAGAATVLLPGGEVYPALERGVIDAADFVGPAVNYNLGFHQVTKYIIMGPPETPAIHQPVDLADITLNLNRWRAVPKNLQERFEAAVHEWSWVHYAGIQKANLEAWPKYRAAGVQIIRLSTVDVRKFRRVAIPIWFKWAKQDKYAKEAFQSQLEYMKALGYVTDVDLRGLSL

SEQ ID NO: 118 - protein, 337 aa, Artificial Sequence
  tsLacBP4  (with signal peptide replaced with M)
MTARGVRWRMQSAWQPGTIGYRTFETWARSIQELTSGELSIEPFPAGAVAGTFEMADAVRSGVLDGMNWFTVYWPGKMPAGVFMSAYPMALSLPHHWDMMFDSFGGRQIVDELYDRQGLVFLGHVQHDLNLIHSKVPLRSFDDFRGKRIRFPGGIIAETFAKVGVRTTLLPGGDVYPALERGTIDAADFVGPAVNYDLGFHQVADYIIMGPPSTPALHQPVDLMDISVNKRSWSRISEHTQKLMYKFVKAYSAEHFAAIQKANHEAWPKYKEAGVEVIHLSEEDAARFREAAIPLWFEWANKDRDAARLFKVHLEVMQDPSVAVITPDDIKDYKLNF

SEQ ID NO: 119 - protein, 337 aa, Artificial Sequence
  rdLacBP5  (with signal peptide replaced with M)
MAAGEGTTWKIQTSHTGGIGLATFKDWASSIEEKTGGELAFTAFGANDVVGDFQLYDAVKNGVLDAVNPFTIYAQGIIPAATFLTSYPLGLRNPHEWDVFFYSLGGLEIARELYAAQGMKFVGPVHHGPNIIHSKVPIRSIDDFAGLKMRMPGGMVAEVFSEIGAETTVLPGSEIFPALEKGTIDAADFVGPAVNYALGFSQVTNYISMGPAGFMSLYQPVDLMDITVGQTAWDALSPQMQQFVEMETHVYSDMHHAAIQKADQEAWAKFEADGTEVTRLSQDDVELMTEVAVPIWFDYANRDKDAARVFKIQLDYMMSGSLGYVTPEQIEGLTLNL

SEQ ID NO: 120 - protein, 332 aa, Artificial Sequence
  msLacBP6  (with signal peptide replaced with M)
MATTWKIQSVWDAGTVGYDLFKEWCDGMEEKTGGELKFTCFPAKAVAADNNGLFDAVRNGVLQGMNPFTLYWSGKIPASVFLSSYPAGPDQPHQWDTMFYSLGMLEKTREIYKKFGLFYVGPIQHDANIIHSKQPINSLDDLKGLKMRLPGGMVAEVFAKFGVAAVSLPGSDIFPALEKGTIDAADYVGPAVNWELGFSQVTKYILMGPPGIMSVYQPVDLMDLTVNLRAWNALDPKLQQIVEDEVRIYSQKHYLAIQKRNIEAMKKFEAAGTTVTRLSQEDLQEFRRAAIPIWYSWANKDEDAREIFDMQLEYMMNDTVGYITEDDIKGMN

SEQ ID NO: 121 - protein, 333 aa, Artificial Sequence
  tsLacBP7  (with signal peptide replaced with M)
MQAPRFRWRIQSAWDAGTVGYTLFQRFAERVKELTDGQIEIQTFPAGAVVGTFDMFDAVKTGVLDGMHPFTLYWAGRMPVTAFLSSYPLGLDRPDQWETWYYALGGLDLARRAFEEQGLFYVGPVQHDYNLIHSKKPIKSFEDFKGVKLRVPGGMIADVFSAAGAATVLLPGGEVYPALERGVIDAADFVGPAVNYNLGFHQVTKYIIMGPPETPAIHQPVDLADITLNLSRWRAVPKNLQERFEAAVHEWSWIHYAGIQKANLETWPKYKAAGVQIIRLTTVDVRKFRRVAIPIWFKWAKQDKYAREAFASQLEYMKALGYVTDADVRGLSL

SEQ ID NO: 122 - protein, 333 aa, Artificial Sequence
  maLacBP8  (with signal peptide replaced with M)
MQAATTWKIQSTWDAGTVGYTLFEEWAKSIEAKSGGELKFQAFPAKAVAADNNALFDAVRNGVLQGMNPFTLYWAGKIPASVFLSSYPAGPDQPHQWDTMFYSMGMLEKTREIYKKFGLFYVGPIQHDANIIHSKQPVNSLDDLKGMKIRVPGGMVAEVFQQFGVSTVSLPGSDIFPALEKGTIDAADFVGPAVNYELGFSQVTDYIIFGPPGVMSIYQPVDLMDLTVSLRAWNSISPELQQLVEDEVRIYSQKHYLAIQARNIEAMEKFKADGDTVTRLSQEDLETWRKAAIPIWFNWANKNDDARAILDIQLKYMMNDTVGYITEEDIKGF

SEQ ID NO: 123 - protein, 344 aa, Artificial Sequence
  adLacBP9  (with signal peptide replaced with M)
MQAPITLRFQSTWPQKDIFHEFALDYAKKVNEMSGGRLKIEVLAAGSVVKAFDLLDAVSKGTLDGGHGVVAYWYGKNTALALWGSGPAFGMDPNMVLAWHHYGGGRQLLEEIYRSLNLDVVSLMYGPMPTQPLGWFKQKPIAKPDDMKGLKFRTVGLSIDIFNGLGAAVNALPGAEIVPAMDRGLLDAAEFNNASSDRVLGFPDVSKIAMLQSFHQASEQFEILFNGKRFQALPADLKSIISIAAQAASADMSWKAIDRYSSDYFEMRDKQGVKFYSTRPEILKRQLEIWDQVMEKRAAENPTFKKVLESQRRFAQRAARWQNDTNVDFKMAYNHFFGGKKKAT

SEQ ID NO: 124 - protein, 316 aa, Artificial Sequence
  pgLacBP10  (with signal peptide replaced with M)
MQEAVEWRMQALWDAGTTPFEFEKKFVERVGELTEGRFKITLYSAGQIVPANQAFDAVRSGAFEMMKTFDGYEAGKIPAFAFTSTIPFGFPQSDQYEAWFYELGGLDLAREAYAKGGLFYIAPTVYGEEPMHSTVKIESIADMAGKKGRFVGLASAVMADLGVAVSPLATAEVYTALEKGLIDFADRGDLTANYEAGLGEVAKFIILPGVHQPTTATSYVANQAAYQKLPDGFKAALAVAAREISGSLRQHILVQDMEVLTKYKDQGVEVVRLDAADIAAARAKAVESWEKATKGDELATRVLKGQVDFMTSLGLL

SEQ ID NO: 125 - protein, 336 aa, Artificial Sequence
  psLacBP11  (with signal peptide replaced with M)
MQQAAGEPAKTYHWKMVTAWPKNYPGLGTSAERLAERVNAMSGGRLTIKVYAAGELVPALEVFDAVSRGTAELGHGASYYWKGKVPTAQFFTSVPFGLSTSEMNAWLSKGGGQAFWDEAYAPFGVKPLVIGNTGMQMGGWYNKEINSLTDLKGLKIRMPGLGGEVLSRLGATTVNLPGGEVFTALQTGAIDATDWVSPYNDLAFGLHKAARYYYYPGWQEPQAVLELLINQKAFDSLPADLQAIVTEASLAASRDMHDDYVYNNALALEQLKQQGTELKRFPDEVLAAMREQSDLILGELAAQSELNGRIWASMKAFQAQVEPMHEISEKELYNWR

SEQ ID NO: 126 - protein, 342 aa, Artificial Sequence
  rsLacBP12  (with signal peptide replaced with M)
MQAPLVMKMQTSWPASDIWMDFAREYVTRVEEMSGGRIKVDLLPAGAVVGAFQVMDAVHDGVIDASHSVSAYWYGKSKAASFFGTGPVFGGSATTMLGWFYQGGGQDLYRELTQDILGMNIVGFYGFPMPAQPFGWFKTEVNGVADIQGFKYRTVGLAADLLQAMGMSVAQLPGGEIVPAMERGVIDAFEFNNPSSDMRFGAQDVAKNYYLSSYHQASESFEYTFNRDFYEDLDPDLQAILKYAVEAASTSNTALALRQYSADLATLAAENGVAVHRTPKDILSGQLEAWDKLIVDLEADEFFKKVLDSQRAWVEQVSYYELMNAADLGLAYEHHFPGKLKL

SEQ ID NO: 127 - protein, 336 aa, Artificial Sequence
  fsLacBP13  (with signal peptide replaced with M)
MEKKIRWKLAMTWGPTLHPLSDTAEHMAEIVKELSDGNFVINIDASNVHKAPFGIFDMVKLGQYEMGHTASYYYKGKNIAFLPLTTMPFGMTAPEQYAWFYYGGGLELMQEAYTKHGMLAFPGGNTGNQMGGWFTKEINSLDDLKGLKMRIPGFAGQIMSKLGVTVTNIPPGELYTALERGTVDAVEWTGPGMDINMGFHKIAKYYYTGWHEPGSEVEFLINEKEYNKLPEKYKKILKIAMKTAAYDMYIQSYEMNAEAWQQMKEKYPDIKVKVFPEEVLKEMKTAYDNLVASYEKESPMFKKIMESKRAYLDKVRDWTHISDYLYLKSTSESNLN

SEQ ID NO: 128 - protein, 331 aa, Artificial Sequence
  taLacBP14  (with signal peptide replaced with M)
MEEYKFKMATFYLKGDSAFDVIDHFRQLVWKKTGGKVRIDAFQAGELGFPVTEILEATSRGVVEMSIFYPNYKAAQDPVMALAGGRPGPMFDLRDQKAQVDATKDLLERSFGRFGVRYIAPMVYGEPEILVSRRPMSSLKDLKGRIFRASGMAAEFYTAIGAQAMMLPAGELYQALQLGTIDGLEWTDYTANYKLGFHEVAKNVLEPTKGVNLHSEATVHAFLVVNPKVWEKLPKEHQKAIQEAADEAYKWGADHLAKLNKTYKDKWIKAGAKVTQLPKEDQDKVIEVSAKILSGYSAKSPDAKEYARRLVELWKKLGYTKWSDALAKQIK

SEQ ID NO: 129 - protein, 5 aa, Artificial Sequence
  Conserved sequence.
  misc_feature (3)..(3): Xaa can be any naturally occurring amino acid
  misc_feature (5)..(5): Xaa can be any naturally occurring amino acid
FTXYX

SEQ ID NO: 130 - protein, 6 aa, Artificial Sequence
  Conserved sequence
  misc_feature (2)..(2): Xaa can be any naturally occurring amino acid
NXIHSK

SEQ ID NO: 131 - protein, 5 aa, Artificial Sequence
  Conserved sequence
  misc_feature (2)..(2): Xaa can be any naturally occurring amino acid
RXPGG

SEQ ID NO: 132 - protein, 4 aa, Artificial Sequence
  Conserved sequence
  misc_feature (4)..(4): Xaa can be any naturally occurring amino acid
LPGX

SEQ ID NO: 133 - protein, 6 aa, Artificial Sequence
  Conserved sequence
VGPAVN

SEQ ID NO: 134 - protein, 5 aa, Artificial Sequence
  Conserved sequence
QPVDL

SEQ ID NO: 135 - DNA, 1400 bp, Artificial Sequence
  Exemplary taLacBP14.186C expression sequence.
cggtcacgcttgggactgccataggctggcccggtgatgccggccacgatgcgtccggcgtagaggatcgagatctcgatcccgcgaaattaatacgactcactatagggagaccacaacggtttccctctagaaataattttgtttaactttaagaaggagatataccatggaagaatataaatttaaaatggcaactttttacctgaaaggtgatagcgcctttgacgtgatcgaccactttcgccaactggtctggaagaaaaccggtggtaaggtacgcatcgatgcgttccaagctggggaactgggctttccagtgaccgagatcctggaagcgaccagtcgtggtgtggtggagatgagcatcttctacccgaactacaaagcggcacaggatccggtgatggccttagcgggaggacgtccgggtccaatgttcgacctgcgtgatcagaaagcccaagtggatgcgaccaaagatctcctggaaaggtccttcggtcgtttcggagttcgctacattgcgcctatggtgtacggtgaaccggagatcctggtctcgagacgtccgatgagtagcctcaaagacctgaaagggcgtatcttccgtgcgagtggtatggcagcggagttctacaccgcaattggcgcacaagcgatgatgcttccagcaggtgagctctaccaggcactgcagttaggcaccatcgatggtctggagtgcaccgactataccgcgaactacaagcttggcttccacgaagtggcgaagaacgtgctggaaccgacgaaaggtgtgaacctccattcggaagctaccgttcatgcgttcctggttgtgaacccgaaagtctgggagaaactgccgaaggaacaccagaaagcgatccaggaagcggcggacgaagcgtacaaatggggtgcggatcaccttgcgaaactgaacaaaacctacaaggacaaatggatcaaagcgggtgcgaaggtgacccaactgccgaaagaagaccaggacaaagtgatcgaagtgtcggcaaagatcctgtctggctatagcgcgaagagtccggatgcgaaagagtacgcgcgtcgtctagtggagctgtggaagaaactgggctacaccaaatggtctgatgcattagcaaaacagattaaaggcggcagccatcatcatcatcatcattaataatgaaagggcgatatccagcacactggcggccgttactagtggatccggctgctaacaaagcccgaaaggaagctgagttggctgctgccaccgctgagcaataactagcataaccccttggggcctctaaacgggtcttgaggggttttttgctgaaaggaggaactatatccggagcgactcccacggcacgttggcaagctcg

SEQ ID NO: 136 - DNA, 1433 bp, Artificial Sequence
  Exemplary rsLacBP12 expression sequence.
cggtcacgcttgggactgccataggctggcccggtgatgccggccacgatgcgtccggcgtagaggatcgagatctcgatcccgcgaaattaatacgactcactatagggagaccacaacggtttccctctagaaataattttgtttaactttaagaaggagatataccatgcaagcaccgttagttatgaaaatgcaaactagttggccagctagcgatatctggatggacttcgcacgtgagtacgtgaccagagtggaagagatgtcaggtggacgcatcaaggtggatctgctgccagcaggtgcggtagttggtgcgttccaggtgatggacgcagtacacgatggggtcatcgatgctagccactcggtgagcgcttactggtatggcaagagcaaagcggctagcttctttggcactggtccagtctttggcggtagtgcaaccacgatgctcggctggttctaccaaggtggaggtcaggacctgtaccgtgaactgacgcaagacatcctcggaatgaacatcgtaggcttctacggtttcccgatgccggcacagccattcggctggttcaagacggaagtgaacggcgttgcggacatccaaggcttcaagtaccgtaccgttggactggcagcagatctgctgcaggctatgggcatgtcagtggcacagctgccaggtggcgaaatcgttccggcaatggagcgtggtgtgatcgatgcgttcgagttcaacaaccctagctcggatatgcgctttggtgcacaagatgtggcgaagaactactacctgtcctcctaccatcaggcatctgagagcttcgagtacaccttcaatcgcgacttctacgaggatctggatcctgacctgcaagccatcctgaagtacgctgtggaagcagcgagtaccagcaataccgcgttagcgctgaggcagtatagcgcagatcttgcgacgttagcggctgaaaacggtgttgcagtgcatcggactccgaaagacatcctgtctggtcagctggaagcatgggacaagctgatcgtggatctcgaagcggatgagttcttcaagaaagtgctggattcccaacgtgcatgggtcgaacaggtctcctactacgagctgatgaacgcagcggatcttggactggcatacgaacatcattttccaggaaaattaaaactgggcggcagccatcatcatcatcatcattaataatgaaagggcgatatccagcacactggcggccgttactagtggatccggctgctaacaaagcccgaaaggaagctgagttggctgctgccaccgctgagcaataactagcataaccccttggggcctctaaacgggtcttgaggggttttttgctgaaaggaggaactatatccggagcgactcccacggcacgttggcaagctcg

SEQ ID NO: 137 - protein, 330 aa, Artificial Sequence
  2ZZV seed sequence (ttLacBP1)
RRYRWRIQTAWDAGTVGYSLFQKFTERVKELTDGQLEVQPFPAGAVVGTFDMFDAVKTGVLDGMNPFTLYWAGRMPVTAFLSSYALGLDRPDQWETWFYSLGGLDIARRAFAEQGLFYVGPVQHDLNIIHSKKPIRRFEDFKGVKLRVPGGMIAEVFAAAGASTVLLPGGEVYPALERGVIDAADFVGPAVNYNLGFHQVAKYIIMGPPETPAIHQPVDLMDFTINLNRWRSLPKPLQERFIAAVHEYSWIHYAGIQKANLEAWPKYRQAGVEVIRLSNEDVRKFRRLAIPIWFKWAKMDKYSREAFASQLEYMKGIGYVTDEELKGLSL

SEQ ID NO: 138 - protein, 109 aa, Escherichia coli
MSDKIIHLTDDSFDTDVLKADGAILVDFWAEWCGPCKMIAPILDEIADEYQGKLTVAKLNIDQNPGTAPKYGIRGIPTLLLFKNGEVAATKVGALSKGQLKEFLDANLA

SEQ ID NO: 139 - protein, 118 aa, Artificial Sequence
  Adaptor0
MSAKIIHLTDDSFDTDVLKADGAILVAFWAEWCGPCKMIAPILDEIADEYQGKLTVAMLNIDQNPGTAPKYGIRGIPTLLLFKNGEVAATKVGALSKGQLKEFLDANLAGGSHHHHHH

SEQ ID NO: 140 - protein, 118 aa, Artificial Sequence
  Adaptor1.0
MSAKIIHLTDDSFDTDVLKADGAILVAFWAEWCGPCKMIAPILDEIADEYQGKLTVAMLNIDQNPGTAPKYGICGIPTLLLFKNGEVAATKVGALSKGQLKEFLDANLAGGSHHHHHH

SEQ ID NO: 141 - protein, 118 aa, Artificial Sequence; identical to SEQ ID NO: 140
  Adaptor2.0a

SEQ ID NO: 142 - protein, 118 aa, Artificial Sequence; identical to SEQ ID NO: 140
  Adaptor2.0b

SEQ ID NO: 143 - protein, 118 aa, Artificial Sequence
  Adaptor3.0
MSAKIIHLTDCSFDTDVLKADGAILVAFWAEWCGPCKMIAPILDEIADEYQGKLTVAMLNIDQNPGTAPKYGIRGIPTLLLFKNGEVAATKVGALSKGQLKEFLDANLAGGSHHHHHH

SEQ ID NO: 144 - protein, 118 aa, Artificial Sequence
  Adaptor4.0
MSAKIIHLTDDSFDCDVLKADGAILVAFWAEWCGPCKMIAPILDEIADEYQGKLTVAMLNIDQNPGTAPKYGIRGIPTLLLFKNGEVAATKVGALSKGQLKEFLDANLAGGSHHHHHH

SEQ ID NO: 145 - protein, 118 aa, Artificial Sequence
  Adaptor5.0
MSAKIIHLTDDSFDTDVLKACGAILVAFWAEWCGPCKMIAPILDEIADEYQGKLTVAMLNIDQNPGTAPKYGIRGIPTLLLFKNGEVAATKVGALSKGQLKEFLDANLAGGSHHHHHH

SEQ ID NO: 146 - protein, 118 aa, Artificial Sequence
  Adaptor6.0
MSAKIIHLTDDSFDTDVLKADGAILVAFWAECCGPCKMIAPILDEIADEYQGKLTVAMLNIDQNPGTAPKYGIRGIPTLLLFKNGEVAATKVGALSKGQLKEFLDANLAGGSHHHHHH

SEQ ID NO: 147 - protein, 118 aa, Artificial Sequence
  Adaptor7.0
MSAKIIHLTDDSFDTDVLKADGAILVAFWAEWCGPCKCIAPILDEIADEYQGKLTVAMLNIDQNPGTAPKYGIRGIPTLLLFKNGEVAATKVGALSKGQLKEFLDANLAGGSHHHHHH

SEQ ID NO: 148 - protein, 118 aa, Artificial Sequence
  Adaptor8.0
MSAKIIHLTDDSFDTDVLKADGAILVAFWAEWCGPCKMIAPILDCIADEYQGKLTVAMLNIDQNPGTAPKYGIRGIPTLLLFKNGEVAATKVGALSKGQLKEFLDANLAGGSHHHHHH

SEQ ID NO: 149 - protein, 118 aa, Artificial Sequence
  Adaptor9.0
MSAKIIHLTDDSFDTDVLKADGAILVAFWAEWCGPCKMIAPILDEIADEYQGCLTVAMLNIDQNPGTAPKYGIRGIPTLLLFKNGEVAATKVGALSKGQLKEFLDANLAGGSHHHHHH

SEQ ID NO: 150 - protein, 118 aa, Artificial Sequence
  Adaptor10.0
MSAKIIHLTDDSFDTDVLKADGAILVAFWAEWCGPCKMIAPILDEIADEYQGKLTVAMLNIDCNPGTAPKYGIRGIPTLLLFKNGEVAATKVGALSKGQLKEFLDANLAGGSHHHHHH

SEQ ID NO: 151 - protein, 118 aa, Artificial Sequence
  Adaptor11.0
MSAKIIHLTDDSFDTDVLKADGAILVAFWAEWCGPCKMIAPILDEIADEYQGKLTVAMLNIDQNPGTAPKCGIRGIPTLLLFKNGEVAATKVGALSKGQLKEFLDANLAGGSHHHHHH

SEQ ID NO: 152 - protein, 118 aa, Artificial Sequence
  Adaptor12.0
MSAKIIHLTDDSFDTDVLKADGAILVAFWAEWCGPCKMIAPILDEIADEYQGKLTVAMLNIDQNPGTAPKYGIRGIPTLLLFKNGECAATKVGALSKGQLKEFLDANLAGGSHHHHHH

SEQ ID NO: 153 - protein, 118 aa, Artificial Sequence
  Adaptor13.0
MSAKIIHLTDDSFDTDVLKADGAILVAFWAEWCGPCKMIAPILDEIADEYQGKLTVAMLNIDQNPGTAPKYGIRGIPTLLLFKNGEVAATKCGALSKGQLKEFLDANLAGGSHHHHHH

SEQ ID NO: 154 - protein, 118 aa, Artificial Sequence
  Adaptor14.0
MSAKIIHLTDDSFDTDVLKADGAILVAFWAEWCGPCKMIAPILDEIADEYQGKLTVAMLNIDQNPGTAPKYGIRGIPTLLLFKNGEVAATKVGALSCGQLKEFLDANLAGGSHHHHHH

SEQ ID NO: 155 - protein, 118 aa, Artificial Sequence
  Adaptor15.0
MSAKIIHLTDDSFDTDVLKADGAILVAFWAEWCGPCKMIAPILDEIADEYQGKLTVAMLNIDQNPGTAPKYGIRGIPTLLLFKNGEVAATKVGALSKGCLKEFLDANLAGGSHHHHHH

SEQ ID NO: 156 - protein, 118 aa, Artificial Sequence
  Adaptor16.0
MSAKIIHLTDDSFDTDVLKADGAILVAFWAEWCGPCKMIAPILDEIADEYQGKLTVAMLNIDQNPGTAPKYGIRGIPTLLLFKNGEVAATKVGALSKGQLKEFLDCNLAGGSHHHHHH